European Patent Application EP 4 134 674 A1, published February 15, 2023. Title: Methods and reagents for detecting an antibody to a Ses iPR-10 allergen. Applicant: EUROIMMUN Medizinische Labordiagnostika AG. Application EP. The sequence listing filed with the application follows.

SEQUENCE LISTING (28 sequences)

SEQ ID NO: 1 - protein, 191 aa, synthetic construct
  REGION 1..36: note = X can be any naturally occurring amino acid or no amino acid
  REGION 37..39: note = X can be any naturally occurring amino acid
  REGION 41..46: note = X can be any naturally occurring amino acid
  SITE 48: note = X can be a polar and/or charged amino acid
  SITE 50: note = X can be any naturally occurring amino acid or no amino acid
  SITE 51: note = X can be any naturally occurring amino acid
  SITE 52: note = X can be a hydrophobic amino acid including glycine, alanine and methionine
  SITE 53: note = X can be any naturally occurring amino acid
  SITE 54: note = X can be a polar and/or charged amino acid
  SITE 55: note = X can be a hydrophobic amino acid including glycine, alanine and methionine
  REGION 56..58: note = X can be any naturally occurring amino acid
  SITE 59: note = X can be a polar and/or charged amino acid
  SITE 61: note = X can be any naturally occurring amino acid
  SITE 62: note = X can be a polar and/or charged amino acid
  REGION 63..65: note = X can be any naturally occurring amino acid
  SITE 66: note = X can be a hydrophobic amino acid including glycine, alanine and methionine
  SITE 67: note = X can be a polar and/or charged amino acid
  REGION 68..69: note = X can be any naturally occurring amino acid
  SITE 71: note = X can be any naturally occurring amino acid
  SITE 72: note = X can be a polar and/or charged amino acid
  SITE 73: note = X can be a hydrophobic amino acid including glycine, alanine and methionine
  SITE 74: note = X can be a polar and/or charged amino acid
  REGION 75..76: note = X can be any naturally occurring amino acid
  SITE 77: note = X can be a polar and/or charged amino acid
  SITE 78: note = X can be any naturally occurring amino acid
  REGION 79..80: note = X can be a polar and/or charged amino acid
  SITE 81: note = X can be a hydrophobic amino acid including glycine, alanine and methionine
  REGION 82..84: note = X can be any naturally occurring amino acid
  SITE 86: note = X can be a polar and/or charged amino acid
  REGION 87..88: note = X can be a hydrophobic amino acid including glycine, alanine and methionine
  SITE 89: note = X can be any naturally occurring amino acid
  SITE 91: note = X can be any naturally occurring amino acid
  SITE 92: note = X can be any naturally occurring amino acid or no amino acid
  SITE 93: note = X can be any naturally occurring amino acid
  SITE 94: note = X can be a hydrophobic amino acid including glycine, alanine and methionine
  REGION 95..97: note = X can be any naturally occurring amino acid
  SITE 98: note = X can be a hydrophobic amino acid including glycine, alanine and methionine
  REGION 99..100: note = X can be a polar and/or charged amino acid
  SITE 101: note = X can be a hydrophobic amino acid including glycine, alanine and methionine
  REGION 102..104: note = X can be any naturally occurring amino acid
  SITE 105: note = X can be a hydrophobic amino acid including glycine, alanine and methionine
  SITE 106: note = X can be a polar and/or charged amino acid
  SITE 107: note = X can be a hydrophobic amino acid including glycine, alanine and methionine
  REGION 108..111: note = X can be any naturally occurring amino acid
  REGION 112..113: note = X can be any naturally occurring amino acid or no amino acid
  SITE 114: note = X can be any naturally occurring amino acid
  SITE 115: note = X can be a hydrophobic amino acid including glycine, alanine and methionine
  SITE 116: note = X can be any naturally occurring amino acid
  SITE 117: note = X can be a polar and/or charged amino acid
  SITE 118: note = X can be a hydrophobic amino acid including glycine, alanine and methionine
  SITE 119: note = X can be any naturally occurring amino acid
  SITE 120: note = X can be a polar and/or charged amino acid
  REGION 121..122: note = X can be any naturally occurring amino acid
  SITE 123: note = X can be a polar and/or charged amino acid
  REGION 124..126: note = X can be any naturally occurring amino acid or no amino acid
  REGION 127..132: note = X can be any naturally occurring amino acid
  SITE 133: note = X can be a hydrophobic amino acid including glycine, alanine and methionine
  SITE 134: note = X can be any naturally occurring amino acid
  REGION 135..137: note = X can be a polar and/or charged amino acid
  SITE 138: note = X can be a hydrophobic amino acid including glycine, alanine and methionine
  SITE 139: note = X can be a polar and/or charged amino acid
  SITE 140: note = X can be any naturally occurring amino acid
  SITE 143: note = X can be a polar and/or charged amino acid
  SITE 144: note = X can be any naturally occurring amino acid
  SITE 145: note = X can be a hydrophobic amino acid including glycine, alanine and methionine
  REGION 146..147: note = X can be any naturally occurring amino acid
  REGION 148..149: note = X can be a hydrophobic amino acid including glycine, alanine and methionine
  SITE 150: note = X can be any naturally occurring amino acid
  SITE 151: note = X can be a hydrophobic amino acid including glycine, alanine and methionine
  SITE 152: note = X can be any naturally occurring amino acid
  SITE 153: note = X can be a polar and/or charged amino acid
  REGION 154..156: note = X can be any naturally occurring amino acid
  REGION 157..191: note = X can be any naturally occurring amino acid or no amino acid
  source 1..191: note = general Ses iPR10 antigenic consensus sequence
XXXXXXXXXXXXXXXXXXXXXXXXXXXXXXXXXXXXXXXKXXXXXXGXGXXXXXXXXXXFXXXXXXXXXKXXXXXXXXXXXXXXYXXXXGXXXXXXXXXXXXXXXXXXXXXXXXXXXXXXXXXXXXXXXXXXXXXXXXXXGKXXXXXXXXXXXXXXXXXXXXXXXXXXXXXXXXXXXXXXXXXXXXXXXXX

SEQ ID NO: 2 - protein, 159 aa, synthetic construct
  source 1..159: note = Ses iPR10-2, antigenic sequence to which antibody binds
GVLTFTEEHTSAVSPSRIFKASILDANNLIPKLLPQVIKSMEFIQGTGSPGSIKQICFAEGSTLSSLKYRIDELNEETYTYNYTVIEGDALTDKLEKITHEVKLEAAPGGGTFSKVTSTYYTKGDFALKEEDVKAGKERVLGVYKVVEAYLLNNPDAYA

SEQ ID NO: 3 - protein, 161 aa, synthetic construct
  source 1..161: note = Ses iPR10-3, antigenic sequence to which antibody binds
GVTSITQEFSSPVAPERLFKALILDSNNLIPKLLPQSIKSVDLLRGDGGAGSIEQVNFTETSHFKYVKHQINELDKQNLVCKYTMIEGDALGDKLESIVYEIKFEASDINGAGCVCKMTSEYHTLGGYEVKEEEIKGGKESAMGIYKVVEAHLLENPHLYA

SEQ ID NO: 4 - protein, 159 aa, synthetic construct
  source 1..159: note = Ses iPR10-4, antigenic sequence to which antibody binds
GVIKVSQSFRTKVTPSRMFKALILDSHNLCPQLMFSSIKSIDFLQGKGEPGTIKQMNFTDASPFNYVKHRIDEMDEEKFMCKYTFIEGDALMDKLDHITYEVKFEPYGFGGCICRITSEYYTKENVEIKEEDIELGKDRAIGMYEVVEAYLLAHPHAYN

SEQ ID NO: 5 - protein, 155 aa, synthetic construct
  source 1..155: note = Ses iPR10-5, antigenic sequence to which antibody binds
GAITYDIEIPSSIPAAKMFKAVVLDADTLIPKIMPQAIKNVEILEGDGGVGTVKIIHFGEGSQYKSAKHRVDAIDTENLTHSYTIVEGDALAGVLESITYHVKIVPTEDGGCICKNRSIYHTKGDVEITEEKIKEGKEKAMQMLKAIEAYLQANA

SEQ ID NO: 6 - protein, 159 aa, synthetic construct
  source 1..159: note = Ses iPR10-6, antigenic sequence to which antibody binds
GVLNYEDELISPVPPARLFKSLVLDGDNLIPKLLPHAFKSFQILEGHGGPGTIKLVTFADGSPYKTAKHRIDEIDEENYIYKYSVIGGDALGEDFDSMTHGFKIEVGADGGSICKTTSTFHTKGEDHVIQEKIKAGKERAKAIFKAVETHLHAHPHEYN

SEQ ID NO: 7 - protein, 179 aa, synthetic construct
  source 1..179: note = Ses iPR10-2, His tagged sequence, prescission protease cleavage site and linker, as used in examples
MSHHHHHHHHLEVLFQGPSMGVLTFTEEHTSAVSPSRIFKASILDANNLIPKLLPQVIKSMEFIQGTGSPGSIKQICFAEGSTLSSLKYRIDELNEETYTYNYTVIEGDALTDKLEKITHEVKLEAAPGGGTFSKVTSTYYTKGDFALKEEDVKAGKERVLGVYKVVEAYLLNNPDAYA

SEQ ID NO: 8 - protein, 181 aa, synthetic construct
  source 1..181: note = Ses iPR10-3, His tagged sequence, prescission protease cleavage site and linker, as used in examples
MSHHHHHHHHLEVLFQGPSMGVTSITQEFSSPVAPERLFKALILDSNNLIPKLLPQSIKSVDLLRGDGGAGSIEQVNFTETSHFKYVKHQINELDKQNLVCKYTMIEGDALGDKLESIVYEIKFEASDINGAGCVCKMTSEYHTLGGYEVKEEEIKGGKESAMGIYKVVEAHLLENPHLYA

SEQ ID NO: 9 - protein, 179 aa, synthetic construct
  source 1..179: note = Ses iPR10-4, His tagged sequence, prescission protease cleavage site and linker, as used in examples
MSHHHHHHHHLEVLFQGPSMGVIKVSQSFRTKVTPSRMFKALILDSHNLCPQLMFSSIKSIDFLQGKGEPGTIKQMNFTDASPFNYVKHRIDEMDEEKFMCKYTFIEGDALMDKLDHITYEVKFEPYGFGGCICRITSEYYTKENVEIKEEDIELGKDRAIGMYEVVEAYLLAHPHAYN

SEQ ID NO: 10 - protein, 179 aa, synthetic construct; identical to SEQ ID NO: 7
  source 1..179: note = Ses iPR10-5, His tagged sequence, prescission protease cleavage site and linker, as used in examples

SEQ ID NO: 11 - protein, 179 aa, synthetic construct
  source 1..179: note = Ses iPR10-6, His tagged sequence, prescission protease cleavage site and linker, as used in examples
MSHHHHHHHHLEVLFQGPSMGVLNYEDELISPVPPARLFKSLVLDGDNLIPKLLPHAFKSFQILEGHGGPGTIKLVTFADGSPYKTAKHRIDEIDEENYIYKYSVIGGDALGEDFDSMTHGFKIEVGADGGSICKTTSTFHTKGEDHVIQEKIKAGKERAKAIFKAVETHLHAHPHEYN

SEQ ID NO: 12 - DNA, 5781 bp, synthetic construct
  source 1..5781: mol_type = other DNA; note = Ses iPR10-2, vector sequence, as used in examples
ggggaattgtgagcggataacaattcccctctagaaataattttgtttaactttaagaaggagatataccatgagccatcatcatcatcatcatcatcatttggaagtgctgtttcagggtccatccatgggtgtactcactttcactgaggagcacacatctgcagtttctccatcaagaatcttcaaagcttcaatcctggacgccaacaacttgatcccaaagcttcttccacaggtcatcaagagcatggaattcattcaaggcactggcagtcctgggagcatcaaacagatctgttttgctgaaggtagcactctgagtagtttgaagtatcggattgatgagctgaatgaagagacatatacgtataattacacagtaattgaaggcgatgcgttgacagacaaacttgagaagatcactcatgaggtgaagttggaggcagcgcccggtggtggcacattctctaaggtgacgagcacgtattacacgaaaggcgattttgctctgaaagaggaagatgttaaagcagggaaggagagggtgcttggggtatacaaggttgttgaggcttacctcctcaacaaccccgatgcctatgcttaatcgagtaagtcgagcaccaccaccaccaccactgagatccggctgctaacaaagcccgaaaggaagctgagttggctgctgccaccgctgagcaataactagcataaccccttggggcctctaaacgggtcttgaggggttttttgctgaaaggaggaactatatccggattggcgaatgggacgcgccctgtagcggcgcattaagcgcggcgggtgtggtggttacgcgcagcgtgaccgctacacttgccagcgccctagcgcccgctcctttcgctttcttcccttcctttctcgccacgttcgccggctttccccgtcaagctctaaatcgggggctccctttagggttccgatttagtgctttacggcacctcgaccccaaaaaacttgattagggtgatggttcacgtagtgggccatcgccctgatagacggtttttcgccctttgacgttggagtccacgttctttaatagtggactcttgttccaaactggaacaacactcaaccctatctcggtctattcttttgatttataagggattttgccgatttcggcctattggttaaaaaatgagctgatttaacaaaaatttaacgcgaattttaacaaaatattaacgtttacaatttcaggtggcacttttcggggaaatgtgcgcggaacccctatttgtttatttttctaaatacattcaaatatgtatccgctcatgaattaattcttagaaaaactcatcgagcatcaaatgaaactgcaatttattcatatcaggattatcaataccatatttttgaaaaagccgtttctgtaatgaaggagaaaactcaccgaggcagttccataggatggcaagatcctggtatcggtctgcgattccgactcgtccaacatcaatacaacctattaatttcccctcgtcaaaaataaggttatcaagtgagaaatcaccatgagtgacgactgaatccggtgagaatggcaaaagtttatgcatttctttccagacttgttcaacaggccagccattacgctcgtcatcaaaatcactcgcatcaaccaaaccgttattcattcgtgattgcgcctgagcgagacgaaatacgcgatcgctgttaaaaggacaattacaaacaggaatcgaatgcaaccggcgcaggaacactgccagcgcatcaacaatattttcacctgaatcaggatattcttctaatacctggaatgctgttttcccggggatcgcagtggtgagtaaccatgcatcatcaggagtacggataaaatgcttgatggtcggaagaggcataaattccgtcagccagtttagtctgaccatctcatctgtaacatcattggcaacgctacctttgccatgtttcagaaacaactctggcgcatcgggcttcccatacaatcgatagattgtcgcacctgattgcccgacattatcgcgagcccatttatacccatataaatcagcatccatgttggaatttaatcgcggcctagagcaagacgtttcccgttgaatatggctcataacaccccttgtattactgtttatgtaagcagacagttttattgttcatgaccaaaatcccttaacgtgagttttcgttccactgagcgtcagaccccgtagaaaagatcaaaggatcttcttgagatcctttttttctgcgcgtaatctgctgcttgcaaacaaaaaaaccaccgctaccagcggtggtttgtttgccggatcaagagctaccaactctttttccgaaggtaactggcttcagcagagcgcagataccaaatactgtccttctagtgtagccgtagttaggccaccacttcaagaactctgtagcaccgcctacatacctcgctctgctaatcctgttaccagtggctgctgccagtggcgataagtcgtgtcttaccgggttggactcaagacgatagttaccggataaggcgcagcggtcgggctgaacggggggttcgtgcacacagcccagcttggagcgaacgacctacaccgaactgagatacctacagcgtgagctatgagaaagcgccacgcttcccgaagggagaaaggcggacaggtatccggtaagcggcagggtcggaacaggagagcgcacgagggagcttccagggggaaacgcctggtatctttatagtcctgtcgggtttcgccacctctgacttgagcgtcgatttttgtgatgctcgtcaggggggcggagcctatggaaaaacgccagcaacgcggcctttttacggttcctggccttttgctggccttttgctcacatgttctttcctgcgttatcccctgattctgtggataaccgtattaccgcctttgagtgagctgataccgctcgccgcagccgaacgaccgagcgcagcgagtcagtgagcgaggaagcggaagagcgcctgatgcggtattttctccttacgcatctgtgcggtatttcacaccgcatatatggtgcactctcagtacaatctgctctgatgccgcatagttaagccagtatacactccgctatcgctacgtgactgggtcatggctgcgccccgacacccgccaacacccgctgacgcgccctgacgggcttgtctgctcccggcatccgcttacagacaagctgtgaccgtctccgggagctgcatgtgtcagaggttttcaccgtcatcaccgaaacgcgcgaggcagctgcggtaaagctcatcagcgtggtcgtgaagcgattcacagatgtctgcctgttcatccgcgtccagctcgttgagtttctccagaagcgttaatgtctggcttctgataaagcgggccatgttaagggcggttttttcctgtttggtcactgatgcctccgtgtaagggggatttctgttcatgggggtaatgataccgatgaaacgagagaggatgctcacgatacgggttactgatgatgaacatgcccggttactggaacgttgtgagggtaaacaactggcggtatggatgcggcgggaccagagaaaaatcactcagggtcaatgccagcgcttcgttaatacagatgtaggtgttccacagggtagccagcagcatcctgcgatgcagatccggaacataatggtgcagggcgctgacttccgcgtttccagactttacgaaacacggaaaccgaagaccattcatgttgttgctcaggtcgcagacgttttgcagcagcagtcgcttcacgttcgctcgcgtatcggtgattcattctgctaaccagtaaggcaaccccgccagcctagccgggtcctcaacgacaggagcacgatcatgcgcacccgtggggccgccatgccggcgataatggcctgcttctcgccgaaacgtttggtggcgggaccagtgacgaaggcttgagcgagggcgtgcaagattccgaataccgcaagcgacaggccgatcatcgtcgcgctccagcgaaagcggtcctcgccgaaaatgacccagagcgctgccggcacctgtcctacgagttgcatgataaagaagacagtcataagtgcggcgacgatagtcatgccccgcgcccaccggaaggagctgactgggttgaaggctctcaagggcatcggtcgagatcccggtgcctaatgagtgagctaacttacattaattgcgttgcgctcactgcccgctttccagtcgggaaacctgtcgtgccagctgcattaatgaatcggccaacgcgcggggagaggcggtttgcgtattgggcgccagggtggtttttcttttcaccagtgagacgggcaacagctgattgcccttcaccgcctggccctgagagagttgcagcaagcggtccacgctggtttgccccagcaggcgaaaatcctgtttgatggtggttaacggcgggatataacatgagctgtcttcggtatcgtcgtatcccactaccgagatatccgcaccaacgcgcagcccggactcggtaatggcgcgcattgcgcccagcgccatctgatcgttggcaaccagcatcgcagtgggaacgatgccctcattcagcatttgcatggtttgttgaaaaccggacatggcactccagtcgccttcccgttccgctatcggctgaatttgattgcgagtgagatatttatgccagccagccagacgcagacgcgccgagacagaacttaatgggcccgctaacagcgcgatttgctggtgacccaatgcgaccagatgctccacgcccagtcgcgtaccgtcttcatgggagaaaataatactgttgatgggtgtctggtcagagacatcaagaaataacgccggaacattagtgcaggcagcttccacagcaatggcatcctggtcatccagcggatagttaatgatcagcccactgacgcgttgcgcgagaagattgtgcaccgccgctttacaggcttcgacgccgcttcgttctaccatcgacaccaccacgctggcacccagttgatcggcgcgagatttaatcgccgcgacaatttgcgacggcgcgtgcagggccagactggaggtggcaacgccaatcagcaacgactgtttgcccgccagttgttgtgccacgcggttgggaatgtaattcagctccgccatcgccgcttccactttttcccgcgttttcgcagaaacgtggctggcctggttcaccacgcgggaaacggtctgataagagacaccggcatactctgcgacatcgtataacgttactggtttcacattcaccaccctgaattgactctcttccgggcgctatcatgccataccgcgaaaggttttgcgccattcgatggtgtccgggatctcgacgctctcccttatgcgactcctgcattaggaagcagcccagtagtaggttgaggccgttgagcaccgccgccgcaaggaatggtgcatgcaaggagatggcgcccaacagtcccccggccacggggcctgccaccatacccacgccgaaacaagcgctcatgagcccgaagtggcgagcccgatcttccccatcggtgatgtcggcgatataggcgccagcaaccgcacctgtggcgccggtgatgccggccacgatgcgtccggcgtagaggatcgagatctcgatcccgcgaaattaatacgactcactata

SEQ ID NO: 13 - DNA, 5787 bp, synthetic construct
  source 1..5787: mol_type = other DNA; note = Ses iPR10-3, vector sequence, as used in examples
ggggaattgtgagcggataacaattcccctctagaaataattttgtttaactttaagaaggagatataccatgagccatcatcatcatcatcatcatcatttggaagtgctgtttcagggtccatccatgggagttacaagcatcactcaagaatttagcagcccggtggcaccggaacgcctgtttaaggccttgatcctagactctaacaacctaataccaaaactcctacctcaatccatcaaaagtgtcgatttactacgaggagatggaggagccggaagcattgagcaagtcaacttcaccgaaactagccattttaagtacgtgaagcatcagataaatgagctggacaaacagaaccttgtgtgcaagtacacgatgattgagggcgatgcattgggcgacaagcttgaatccatcgtgtacgagatcaagtttgaggcatccgacattaatggtgcaggttgtgtgtgcaagatgacgagtgagtaccacacccttggagggtatgaagttaaggaggaagaaatcaagggcgggaaagagagtgcgatgggcatatacaaagttgtggaagctcacctcttggagaatccccatctttatgcttaatcgagtaagtcgagcaccaccaccaccaccactgagatccggctgctaacaaagcccgaaaggaagctgagttggctgctgccaccgctgagcaataactagcataaccccttggggcctctaaacgggtcttgaggggttttttgctgaaaggaggaactatatccggattggcgaatgggacgcgccctgtagcggcgcattaagcgcggcgggtgtggtggttacgcgcagcgtgaccgctacacttgccagcgccctagcgcccgctcctttcgctttcttcccttcctttctcgccacgttcgccggctttccccgtcaagctctaaatcgggggctccctttagggttccgatttagtgctttacggcacctcgaccccaaaaaacttgattagggtgatggttcacgtagtgggccatcgccctgatagacggtttttcgccctttgacgttggagtccacgttctttaatagtggactcttgttccaaactggaacaacactcaaccctatctcggtctattcttttgatttataagggattttgccgatttcggcctattggttaaaaaatgagctgatttaacaaaaatttaacgcgaattttaacaaaatattaacgtttacaatttcaggtggcacttttcggggaaatgtgcgcggaacccctatttgtttatttttctaaatacattcaaatatgtatccgctcatgaattaattcttagaaaaactcatcgagcatcaaatgaaactgcaatttattcatatcaggattatcaataccatatttttgaaaaagccgtttctgtaatgaaggagaaaactcaccgaggcagttccataggatggcaagatcctggtatcggtctgcgattccgactcgtccaacatcaatacaacctattaatttcccctcgtcaaaaataaggttatcaagtgagaaatcaccatgagtgacgactgaatccggtgagaatggcaaaagtttatgcatttctttccagacttgttcaacaggccagccattacgctcgtcatcaaaatcactcgcatcaaccaaaccgttattcattcgtgattgcgcctgagcgagacgaaatacgcgatcgctgttaaaaggacaattacaaacaggaatcgaatgcaaccggcgcaggaacactgccagcgcatcaacaatattttcacctgaatcaggatattcttctaatacctggaatgctgttttcccggggatcgcagtggtgagtaaccatgcatcatcaggagtacggataaaatgcttgatggtcggaagaggcataaattccgtcagccagtttagtctgaccatctcatctgtaacatcattggcaacgctacctttgccatgtttcagaaacaactctggcgcatcgggcttcccatacaatcgatagattgtcgcacctgattgcccgacattatcgcgagcccatttatacccatataaatcagcatccatgttggaatttaatcgcggcctagagcaagacgtttcccgttgaatatggctcataacaccccttgtattactgtttatgtaagcagacagttttattgttcatgaccaaaatcccttaacgtgagttttcgttccactgagcgtcagaccccgtagaaaagatcaaaggatcttcttgagatcctttttttctgcgcgtaatctgctgcttgcaaacaaaaaaaccaccgctaccagcggtggtttgtttgccggatcaagagctaccaactctttttccgaaggtaactggcttcagcagagcgcagataccaaatactgtccttctagtgtagccgtagttaggccaccacttcaagaactctgtagcaccgcctacatacctcgctctgctaatcctgttaccagtggctgctgccagtggcgataagtcgtgtcttaccgggttggactcaagacgatagttaccggataaggcgcagcggtcgggctgaacggggggttcgtgcacacagcccagcttggagcgaacgacctacaccgaactgagatacctacagcgtgagctatgagaaagcgccacgcttcccgaagggagaaaggcggacaggtatccggtaagcggcagggtcggaacaggagagcgcacgagggagcttccagggggaaacgcctggtatctttatagtcctgtcgggtttcgccacctctgacttgagcgtcgatttttgtgatgctcgtcaggggggcggagcctatggaaaaacgccagcaacgcggcctttttacggttcctggccttttgctggccttttgctcacatgttctttcctgcgttatcccctgattctgtggataaccgtattaccgcctttgagtgagctgataccgctcgccgcagccgaacgaccgagcgcagcgagtcagtgagcgaggaagcggaagagcgcctgatgcggtattttctccttacgcatctgtgcggtatttcacaccgcatatatggtgcactctcagtacaatctgctctgatgccgcatagttaagccagtatacactccgctatcgctacgtgactgggtcatggctgcgccccgacacccgccaacacccgctgacgcgccctgacgggcttgtctgctcccggcatccgcttacagacaagctgtgaccgtctccgggagctgcatgtgtcagaggttttcaccgtcatcaccgaaacgcgcgaggcagctgcggtaaagctcatcagcgtggtcgtgaagcgattcacagatgtctgcctgttcatccgcgtccagctcgttgagtttctccagaagcgttaatgtctggcttctgataaagcgggccatgttaagggcggttttttcctgtttggtcactgatgcctccgtgtaagggggatttctgttcatgggggtaatgataccgatgaaacgagagaggatgctcacgatacgggttactgatgatgaacatgcccggttactggaacgttgtgagggtaaacaactggcggtatggatgcggcgggaccagagaaaaatcactcagggtcaatgccagcgcttcgttaatacagatgtaggtgttccacagggtagccagcagcatcctgcgatgcagatccggaacataatggtgcagggcgctgacttccgcgtttccagactttacgaaacacggaaaccgaagaccattcatgttgttgctcaggtcgcagacgttttgcagcagcagtcgcttcacgttcgctcgcgtatcggtgattcattctgctaaccagtaaggcaaccccgccagcctagccgggtcctcaacgacaggagcacgatcatgcgcacccgtggggccgccatgccggcgataatggcctgcttctcgccgaaacgtttggtggcgggaccagtgacgaaggcttgagcgagggcgtgcaagattccgaataccgcaagcgacaggccgatcatcgtcgcgctccagcgaaagcggtcctcgccgaaaatgacccagagcgctgccggcacctgtcctacgagttgcatgataaagaagacagtcataagtgcggcgacgatagtcatgccccgcgcccaccggaaggagctgactgggttgaaggctctcaagggcatcggtcgagatcccggtgcctaatgagtgagctaacttacattaattgcgttgcgctcactgcccgctttccagtcgggaaacctgtcgtgccagctgcattaatgaatcggccaacgcgcggggagaggcggtttgcgtattgggcgccagggtggtttttcttttcaccagtgagacgggcaacagctgattgcccttcaccgcctggccctgagagagttgcagcaagcggtccacgctggtttgccccagcaggcgaaaatcctgtttgatggtggttaacggcgggatataacatgagctgtcttcggtatcgtcgtatcccactaccgagatatccgcaccaacgcgcagcccggactcggtaatggcgcgcattgcgcccagcgccatctgatcgttggcaaccagcatcgcagtgggaacgatgccctcattcagcatttgcatggtttgttgaaaaccggacatggcactccagtcgccttcccgttccgctatcggctgaatttgattgcgagtgagatatttatgccagccagccagacgcagacgcgccgagacagaacttaatgggcccgctaacagcgcgatttgctggtgacccaatgcgaccagatgctccacgcccagtcgcgtaccgtcttcatgggagaaaataatactgttgatgggtgtctggtcagagacatcaagaaataacgccggaacattagtgcaggcagcttccacagcaatggcatcctggtcatccagcggatagttaatgatcagcccactgacgcgttgcgcgagaagattgtgcaccgccgctttacaggcttcgacgccgcttcgttctaccatcgacaccaccacgctggcacccagttgatcggcgcgagatttaatcgccgcgacaatttgcgacggcgcgtgcagggccagactggaggtggcaacgccaatcagcaacgactgtttgcccgccagttgttgtgccacgcggttgggaatgtaattcagctccgccatcgccgcttccactttttcccgcgttttcgcagaaacgtggctggcctggttcaccacgcgggaaacggtctgataagagacaccggcatactctgcgacatcgtataacgttactggtttcacattcaccaccctgaattgactctcttccgggcgctatcatgccataccgcgaaaggttttgcgccattcgatggtgtccgggatctcgacgctctcccttatgcgactcctgcattaggaagcagcccagtagtaggttgaggccgttgagcaccgccgccgcaaggaatggtgcatgcaaggagatggcgcccaacagtcccccggccacggggcctgccaccatacccacgccgaaacaagcgctcatgagcccgaagtggcgagcccgatcttccccatcggtgatgtcggcgatataggcgccagcaaccgcacctgtggcgccggtgatgccggccacgatgcgtccggcgtagaggatcgagatctcgatcccgcgaaattaatacgactcactata

SEQ ID NO: 14 - DNA, 5781 bp, synthetic construct
  source 1..5781: mol_type = other DNA; note = Ses iPR10-4, vector sequence, as used in example
ggggaattgtgagcggataacaattcccctctagaaataattttgtttaactttaagaaggagatataccatgagccatcatcatcatcatcatcatcatttggaagtgctgtttcagggtccatccatgggtgtgatcaaggtgtcccaatccttcagaacaaaagtgaccccaagtaggatgttcaaggccctgatcttggattctcacaacctctgcccccagctcatgttctcctcaatcaagagcatcgacttcctccaaggcaaaggcgagcccggaaccatcaaacagatgaacttcaccgatgctagtccattcaactacgtgaaacataggatcgacgagatggatgaagagaagttcatgtgcaagtacactttcatcgaaggagatgcgttgatggacaagcttgatcacatcacttatgaagtgaagttcgaaccgtatggctttggagggtgtatttgtcggataacaagtgagtattacacaaaagagaatgtggagataaaggaggaagatattgagcttgggaaagatagggctattgggatgtatgaagttgtggaggcctatctcttggcacaccctcatgcctataattaatcgagtaagtcgagcaccaccaccaccaccactgagatccggctgctaacaaagcccgaaaggaagctgagttggctgctgccaccgctgagcaataactagcataaccccttggggcctctaaacgggtcttgaggggttttttgctgaaaggaggaactatatccggattggcgaatgggacgcgccctgtagcggcgcattaagcgcggcgggtgtggtggttacgcgcagcgtgaccgctacacttgccagcgccctagcgcccgctcctttcgctttcttcccttcctttctcgccacgttcgccggctttccccgtcaagctctaaatcgggggctccctttagggttccgatttagtgctttacggcacctcgaccccaaaaaacttgattagggtgatggttcacgtagtgggccatcgccctgatagacggtttttcgccctttgacgttggagtccacgttctttaatagtggactcttgttccaaactggaacaacactcaaccctatctcggtctattcttttgatttataagggattttgccgatttcggcctattggttaaaaaatgagctgatttaacaaaaatttaacgcgaattttaacaaaatattaacgtttacaatttcaggtggcacttttcggggaaatgtgcgcggaacccctatttgtttatttttctaaatacattcaaatatgtatccgctcatgaattaattcttagaaaaactcatcgagcatcaaatgaaactgcaatttattcatatcaggattatcaataccatatttttgaaaaagccgtttctgtaatgaaggagaaaactcaccgaggcagttccataggatggcaagatcctggtatcggtctgcgattccgactcgtccaacatcaatacaacctattaatttcccctcgtcaaaaataaggttatcaagtgagaaatcaccatgagtgacgactgaatccggtgagaatggcaaaagtttatgcatttctttccagacttgttcaacaggccagccattacgctcgtcatcaaaatcactcgcatcaaccaaaccgttattcattcgtgattgcgcctgagcgagacgaaatacgcgatcgctgttaaaaggacaattacaaacaggaatcgaatgcaaccggcgcaggaacactgccagcgcatcaacaatattttcacctgaatcaggatattcttctaatacctggaatgctgttttcccggggatcgcagtggtgagtaaccatgcatcatcaggagtacggataaaatgcttgatggtcggaagaggcataaattccgtcagccagtttagtctgaccatctcatctgtaacatcattggcaacgctacctttgccatgtttcagaaacaactctggcgcatcgggcttcccatacaatcgatagattgtcgcacctgattgcccgacattatcgcgagcccatttatacccatataaatcagcatccatgttggaatttaatcgcggcctagagcaagacgtttcccgttgaatatggctcataacaccccttgtattactgtttatgtaagcagacagttttattgttcatgaccaaaatcccttaacgtgagttttcgttccactgagcgtcagaccccgtagaaaagatcaaaggatcttcttgagatcctttttttctgcgcgtaatctgctgcttgcaaacaaaaaaaccaccgctaccagcggtggtttgtttgccggatcaagagctaccaactctttttccgaaggtaactggcttcagcagagcgcagataccaaatactgtccttctagtgtagccgtagttaggccaccacttcaagaactctgtagcaccgcctacatacctcgctctgctaatcctgttaccagtggctgctgccagtggcgataagtcgtgtcttaccgggttggactcaagacgatagttaccggataaggcgcagcggtcgggctgaacggggggttcgtgcacacagcccagcttggagcgaacgacctacaccgaactgagatacctacagcgtgagctatgagaaagcgccacgcttcccgaagggagaaaggcggacaggtatccggtaagcggcagggtcggaacaggagagcgcacgagggagcttccagggggaaacgcctggtatctttatagtcctgtcgggtttcgccacctctgacttgagcgtcgatttttgtgatgctcgtcaggggggcggagcctatggaaaaacgccagcaacgcggcctttttacggttcctggccttttgctggccttttgctcacatgttctttcctgcgttatcccctgattctgtggataaccgtattaccgcctttgagtgagctgataccgctcgccgcagccgaacgaccgagcgcagcgagtcagtgagcgaggaagcggaagagcgcctgatgcggtattttctccttacgcatctgtgcggtatttcacaccgcatatatggtgcactctcagtacaatctgctctgatgccgcatagttaagccagtatacactccgctatcgctacgtgactgggtcatggctgcgccccgacacccgccaacacccgctgacgcgccctgacgggcttgtctgctcccggcatccgcttacagacaagctgtgaccgtctccgggagctgcatgtgtcagaggttttcaccgtcatcaccgaaacgcgcgaggcagctgcggtaaagctcatcagcgtggtcgtgaagcgattcacagatgtctgcctgttcatccgcgtccagctcgttgagtttctccagaagcgttaatgtctggcttctgataaagcgggccatgttaagggcggttttttcctgtttggtcactgatgcctccgtgtaagggggatttctgttcatgggggtaatgataccgatgaaacgagagaggatgctcacgatacgggttactgatgatgaacatgcccggttactggaacgttgtgagggtaaacaactggcggtatggatgcggcgggaccagagaaaaatcactcagggtcaatgccagcgcttcgttaatacagatgtaggtgttccacagggtagccagcagcatcctgcgatgcagatccggaacataatggtgcagggcgctgacttccgcgtttccagactttacgaaacacggaaaccgaagaccattcatgttgttgctcaggtcgcagacgttttgcagcagcagtcgcttcacgttcgctcgcgtatcggtgattcattctgctaaccagtaaggcaaccccgccagcctagccgggtcctcaacgacaggagcacgatcatgcgcacccgtggggccgccatgccggcgataatggcctgcttctcgccgaaacgtttggtggcgggaccagtgacgaaggcttgagcgagggcgtgcaagattccgaataccgcaagcgacaggccgatcatcgtcgcgctccagcgaaagcggtcctcgccgaaaatgacccagagcgctgccggcacctgtcctacgagttgcatgataaagaagacagtcataagtgcggcgacgatagtcatgccccgcgcccaccggaaggagctgactgggttgaaggctctcaagggcatcggtcgagatcccggtgcctaatgagtgagctaacttacattaattgcgttgcgctcactgcccgctttccagtcgggaaacctgtcgtgccagctgcattaatgaatcggccaacgcgcggggagaggcggtttgcgtattgggcgccagggtggtttttcttttcaccagtgagacgggcaacagctgattgcccttcaccgcctggccctgagagagttgcagcaagcggtccacgctggtttgccccagcaggcgaaaatcctgtttgatggtggttaacggcgggatataacatgagctgtcttcggtatcgtcgtatcccactaccgagatatccgcaccaacgcgcagcccggactcggtaatggcgcgcattgcgcccagcgccatctgatcgttggcaaccagcatcgcagtgggaacgatgccctcattcagcatttgcatggtttgttgaaaaccggacatggcactccagtcgccttcccgttccgctatcggctgaatttgattgcgagtgagatatttatgccagccagccagacgcagacgcgccgagacagaacttaatgggcccgctaacagcgcgatttgctggtgacccaatgcgaccagatgctccacgcccagtcgcgtaccgtcttcatgggagaaaataatactgttgatgggtgtctggtcagagacatcaagaaataacgccggaacattagtgcaggcagcttccacagcaatggcatcctggtcatccagcggatagttaatgatcagcccactgacgcgttgcgcgagaagattgtgcaccgccgctttacaggcttcgacgccgcttcgttctaccatcgacaccaccacgctggcacccagttgatcggcgcgagatttaatcgccgcgacaatttgcgacggcgcgtgcagggccagactggaggtggcaacgccaatcagcaacgactgtttgcccgccagttgttgtgccacgcggttgggaatgtaattcagctccgccatcgccgcttccactttttcccgcgttttcgcagaaacgtggctggcctggttcaccacgcgggaaacggtctgataagagacaccggcatactctgcgacatcgtataacgttactggtttcacattcaccaccctgaattgactctcttccgggcgctatcatgccataccgcgaaaggttttgcgccattcgatggtgtccgggatctcgacgctctcccttatgcgactcctgcattaggaagcagcccagtagtaggttgaggccgttgagcaccgccgccgcaaggaatggtgcatgcaaggagatggcgcccaacagtcccccggccacggggcctgccaccatacccacgccgaaacaagcgctcatgagcccgaagtggcgagcccgatcttccccatcggtgatgtcggcgatataggcgccagcaaccgcacctgtggcgccggtgatgccggccacgatgcgtccggcgtagaggatcgagatctcgatcccgcgaaattaatacgactcactata

SEQ ID NO: 15 - DNA, 5769 bp, synthetic construct
  source 1..5769: mol_type = other DNA; note = Ses iPR10-5, vector sequence, as used in examples
ggggaattgtgagcggataacaattcccctctagaaataattttgtttaactttaagaaggagatataccatgagccatcatcatcatcatcatcatcatttggaagtgctgtttcagggtccatccatgggtgccatcacttacgatattgagattccttcctcaatcccggccgccaagatgtttaaggccgttgtcctcgatgcggatacccttattcctaaaatcatgccccaggctattaaaaacgttgaaatcttggaaggagatggtggtgtgggaactgtcaaaatcatccattttggtgagggcagccagtataagagcgcaaagcaccgtgttgatgctattgacacggagaatttgacccacagctacaccattgttgagggtgacgcactggccggagttcttgaatccatcacttatcatgtcaagattgtgccgactgaagatggaggatgcatatgcaagaacaggagcatttaccacaccaagggcgacgttgagatcaccgaagagaagatcaaggaaggaaaggagaaggcaatgcagatgctcaaggccattgaagcttacctccaagctaatgcctaatcgagtaagtcgagcaccaccaccaccaccactgagatccggctgctaacaaagcccgaaaggaagctgagttggctgctgccaccgctgagcaataactagcataaccccttggggcctctaaacgggtcttgaggggttttttgctgaaaggaggaactatatccggattggcgaatgggacgcgccctgtagcggcgcattaagcgcggcgggtgtggtggttacgcgcagcgtgaccgctacacttgccagcgccctagcgcccgctcctttcgctttcttcccttcctttctcgccacgttcgccggctttccccgtcaagctctaaatcgggggctccctttagggttccgatttagtgctttacggcacctcgaccccaaaaaacttgattagggtgatggttcacgtagtgggccatcgccctgatagacggtttttcgccctttgacgttggagtccacgttctttaatagtggactcttgttccaaactggaacaacactcaaccctatctcggtctattcttttgatttataagggattttgccgatttcggcctattggttaaaaaatgagctgatttaacaaaaatttaacgcgaattttaacaaaatattaacgtttacaatttcaggtggcacttttcggggaaatgtgcgcggaacccctatttgtttatttttctaaatacattcaaatatgtatccgctcatgaattaattcttagaaaaactcatcgagcatcaaatgaaactgcaatttattcatatcaggattatcaataccatatttttgaaaaagccgtttctgtaatgaaggagaaaactcaccgaggcagttccataggatggcaagatcctggtatcggtctgcgattccgactcgtccaacatcaatacaacctattaatttcccctcgtcaaaaataaggttatcaagtgagaaatcaccatgagtgacgactgaatccggtgagaatggcaaaagtttatgcatttctttccagacttgttcaacaggccagccattacgctcgtcatcaaaatcactcgcatcaaccaaaccgttattcattcgtgattgcgcctgagcgagacgaaatacgcgatcgctgttaaaaggacaattacaaacaggaatcgaatgcaaccggcgcaggaacactgccagcgcatcaacaatattttcacctgaatcaggatattcttctaatacctggaatgctgttttcccggggatcgcagtggtgagtaaccatgcatcatcaggagtacggataaaatgcttgatggtcggaagaggcataaattccgtcagccagtttagtctgaccatctcatctgtaacatcattggcaacgctacctttgccatgtttcagaaacaactctggcgcatcgggcttcccatacaatcgatagattgtcgcacctgattgcccgacattatcgcgagcccatttatacccatataaatcagcatccatgttggaatttaatcgcggcctagagcaagacgtttcccgttgaatatggctcataacaccccttgtattactgtttatgtaagcagacagttttattgttcatgaccaaaatcccttaacgtgagttttcgttccactgagcgtcagaccccgtagaaaagatcaaaggatcttcttgagatcctttttttctgcgcgtaatctgctgcttgcaaacaaaaaaaccaccgctaccagcggtggtttgtttgccggatcaagagctaccaactctttttccgaaggtaactggcttcagcagagcgcagataccaaatactgtccttctagtgtagccgtagttaggccaccacttcaagaactctgtagcaccgcctacatacctcgctctgctaatcctgttaccagtggctgctgccagtggcgataagtcgtgtcttaccgggttggactcaagacgatagttaccggataaggcgcagcggtcgggctgaacggggggttcgtgcacacagcccagcttggagcgaacgacctacaccgaactgagatacctacagcgtgagctatgagaaagcgccacgcttcccgaagggagaaaggcggacaggtatccggtaagcggcagggtcggaacaggagagcgcacgagggagcttccagggggaaacgcctggtatctttatagtcctgtcgggtttcgccacctctgacttgagcgtcgatttttgtgatgctcgtcaggggggcggagcctatggaaaaacgccagcaacgcggcctttttacggttcctggccttttgctggccttttgctcacatgttctttcctgcgttatcccctgattctgtggataaccgtattaccgcctttgagtgagctgataccgctcgccgcagccgaacgaccgagcgcagcgagtcagtgagcgaggaagcggaagagcgcctgatgcggtattttctccttacgcatctgtgcggtatttcacaccgcatatatggtgcactctcagtacaatctgctctgatgccgcatagttaagccagtatacactccgctatcgctacgtgactgggtcatggctgcgccccgacacccgccaacacccgctgacgcgccctgacgggcttgtctgctcccggcatccgcttacagacaagctgtgaccgtctccgggagctgcatgtgtcagaggttttcaccgtcatcaccgaaacgcgcgaggcagctgcggtaaagctcatcagcgtggtcgtgaagcgattcacagatgtctgcctgttcatccgcgtccagctcgttgagtttctccagaagcgttaatgtctggcttctgataaagcgggccatgttaagggcggttttttcctgtttggtcactgatgcctccgtgtaagggggatttctgttcatgggggtaatgataccgatgaaacgagagaggatgctcacgatacgggttactgatgatgaacatgcccggttactggaacgttgtgagggtaaacaactggcggtatggatgcggcgggaccagagaaaaatcactcagggtcaatgccagcgcttcgttaatacagatgtaggtgttccacagggtagccagcagcatcctgcgatgcagatccggaacataatggtgcagggcgctgacttccgcgtttccagactttacgaaacacggaaaccgaagaccattcatgttgttgctcaggtcgcagacgttttgcagcagcagtcgcttcacgttcgctcgcgtatcggtgattcattctgctaaccagtaaggcaaccccgccagcctagccgggtcctcaacgacaggagcacgatcatgcgcacccgtggggccgccatgccggcgataatggcctgcttctcgccgaaacgtttggtggcgggaccagtgacgaaggcttgagcgagggcgtgcaagattccgaataccgcaagcgacaggccgatcatcgtcgcgctccagcgaaagcggtcctcgccgaaaatgacccagagcgctgccggcacctgtcctacgagttgcatgataaagaagacagtcataagtgcggcgacgatagtcatgccccgcgcccaccggaaggagctgactgggttgaaggctctcaagggcatcggtcgagatcccggtgcctaatgagtgagctaacttacattaattgcgttgcgctcactgcccgctttccagtcgggaaacctgtcgtgccagctgcattaatgaatcggccaacgcgcggggagaggcggtttgcgtattgggcgccagggtggtttttcttttcaccagtgagacgggcaacagctgattgcccttcaccgcctggccctgagagagttgcagcaagcggtccacgctggtttgccccagcaggcgaaaatcctgtttgatggtggttaacggcgggatataacatgagctgtcttcggtatcgtcgtatcccactaccgagatatccgcaccaacgcgcagcccggactcggtaatggcgcgcattgcgcccagcgccatctgatcgttggcaaccagcatcgcagtgggaacgatgccctcattcagcatttgcatggtttgttgaaaaccggacatggcactccagtcgccttcccgttccgctatcggctgaatttgattgcgagtgagatatttatgccagccagccagacgcagacgcgccgagacagaacttaatgggcccgctaacagcgcgatttgctggtgacccaatgcgaccagatgctccacgcccagtcgcgtaccgtcttcatgggagaaaataatactgttgatgggtgtctggtcagagacatcaagaaataacgccggaacattagtgcaggcagcttccacagcaatggcatcctggtcatccagcggatagttaatgatcagcccactgacgcgttgcgcgagaagattgtgcaccgccgctttacaggcttcgacgccgcttcgttctaccatcgacaccaccacgctggcacccagttgatcggcgcgagatttaatcgccgcgacaatttgcgacggcgcgtgcagggccagactggaggtggcaacgccaatcagcaacgactgtttgcccgccagttgttgtgccacgcggttgggaatgtaattcagctccgccatcgccgcttccactttttcccgcgttttcgcagaaacgtggctggcctggttcaccacgcgggaaacggtctgataagagacaccggcatactctgcgacatcgtataacgttactggtttcacattcaccaccctgaattgactctcttccgggcgctatcatgccataccgcgaaaggttttgcgccattcgatggtgtccgggatctcgacgctctcccttatgcgactcctgcattaggaagcagcccagtagtaggttgaggccgttgagcaccgccgccgcaaggaatggtgcatgcaaggagatggcgcccaacagtcccccggccacggggcctgccaccatacccacgccgaaacaagcgctcatgagcccgaagtggcgagcccgatcttccccatcggtgatgtcggcgatataggcgccagcaaccgcacctgtggcgccggtgatgccggccacgatgcgtccggcgtagaggatcgagatctcgatcccgcgaaattaatacgactcactata

SEQ ID NO: 16 - DNA, 5781 bp, synthetic construct
  source 1..5781: mol_type = other DNA; note = Ses iPR10-6, vector sequence, as used in examples
ggggaattgtgagcggataacaattcccctctagaaataattttgtttaactttaagaaggagatataccatgagccatcatcatcatcatcatcatcatttggaagtgctgtttcagggtccatccatgggtgtgctcaattatgaggatgaactgatctccccagtcccaccagctaggttgtttaagtccctcgttctggacggagacaacctcattcctaagcttctgccacatgcctttaagagctttcaaatcctagagggccatggaggacctggaaccatcaaattggtcacttttgctgatgggagtccttacaagacagcaaagcatcgtattgatgaaattgacgaggaaaattacatatacaagtacagcgtgataggaggtgatgctcttggggaagattttgattccatgacgcacggtttcaagatcgaagtcggggcggatggaggatctatctgcaaaaccaccagcacattccacaccaaaggggaagatcatgttatacaagaaaagatcaaggctggcaaagagagggcaaaggcaattttcaaggctgttgagactcacctccatgcacaccctcatgaatacaactaatcgagtaagtcgagcaccaccaccaccaccactgagatccggctgctaacaaagcccgaaaggaagctgagttggctgctgccaccgctgagcaataactagcataaccccttggggcctctaaacgggtcttgaggggttttttgctgaaaggaggaactatatccggattggcgaatgggacgcgccctgtagcggcgcattaagcgcggcgggtgtggtggttacgcgcagcgtgaccgctacacttgccagcgccctagcgcccgctcctttcgctttcttcccttcctttctcgccacgttcgccggctttccccgtcaagctctaaatcgggggctccctttagggttccgatttagtgctttacggcacctcgaccccaaaaaacttgattagggtgatggttcacgtagtgggccatcgccctgatagacggtttttcgccctttgacgttggagtccacgttctttaatagtggactcttgttccaaactggaacaacactcaaccctatctcggtctattcttttgatttataagggattttgccgatttcggcctattggttaaaaaatgagctgatttaacaaaaatttaacgcgaattttaacaaaatattaacgtttacaatttcaggtggcacttttcggggaaatgtgcgcggaacccctatttgtttatttttctaaatacattcaaatatgtatccgctcatgaattaattcttagaaaaactcatcgagcatcaaatgaaactgcaatttattcatatcaggattatcaataccatatttttgaaaaagccgtttctgtaatgaaggagaaaactcaccgaggcagttccataggatggcaagatcctggtatcggtctgcgattccgactcgtccaacatcaatacaacctattaatttcccctcgtcaaaaataaggttatcaagtgagaaatcaccatgagtgacgactgaatccggtgagaatggcaaaagtttatgcatttctttccagacttgttcaacaggccagccattacgctcgtcatcaaaatcactcgcatcaaccaaaccgttattcattcgtgattgcgcctgagcgagacgaaatacgcgatcgctgttaaaaggacaattacaaacaggaatcgaatgcaaccggcgcaggaacactgccagcgcatcaacaatattttcacctgaatcaggatattcttctaatacctggaatgctgttttcccggggatcgcagtggtgagtaaccatgcatcatcaggagtacggataaaatgcttgatggtcggaagaggcataaattccgtcagccagtttagtctgaccatctcatctgtaacatcattggcaacgctacctttgccatgtttcagaaacaactctggcgcatcgggcttcccatacaatcgatagattgtcgcacctgattgcccgacattatcgcgagcccatttatacccatataaatcagcatccatgttggaatttaatcgcggcctagagcaagacgtttcccgttgaatatggctcataacaccccttgtattactgtttatgtaagcagacagttttattgttcatgaccaaaatcccttaacgtgagttttcgttccactgagcgtcagaccccgtagaaaagatcaaaggatcttcttgagatcctttttttctgcgcgtaatctgctgcttgcaaacaaaaaaaccaccgctaccagcggtggtttgtttgccggatcaagagctaccaactctttttccgaaggtaactggcttcagcagagcgcagataccaaatactgtccttctagtgtagccgtagttaggccaccacttcaagaactctgtagcaccgcctacatacctcgctctgctaatcctgttaccagtggctgctgccagtggcgataagtcgtgtcttaccgggttggactcaagacgatagttaccggataaggcgcagcggtcgggctgaacggggggttcgtgcacacagcccagcttggagcgaacgacctacaccgaactgagatacctacagcgtgagctatgagaaagcgccacgcttcccgaagggagaaaggcggacaggtatccggtaagcggcagggtcggaacaggagagcgcacgagggagcttccagggggaaacgcctggtatctttatagtcctgtcgggtttcgccacctctgacttgagcgtcgatttttgtgatgctcgtcaggggggcggagcctatggaaaaacgccagcaacgcggcctttttacggttcctggccttttgctggccttttgctcacatgttctttcctgcgttatcccctgattctgtggataaccgtattaccgcctttgagtgagctgataccgctcgccgcagccgaacgaccgagcgcagcgagtcagtgagcgaggaagcggaagagcgcctgatgcggtattttctccttacgcatctgtgcggtatttcacaccgcatatatggtgcactctcagtacaatctgctctgatgccgcatagttaagccagtatacactccgctatcgctacgtgactgggtcatggctgcgccccgacacccgccaacacccgctgacgcgccctgacgggcttgtctgctcccggcatccgcttacagacaagctgtgaccgtctccgggagctgcatgtgtcagaggttttcaccgtcatcaccgaaacgcgcgaggcagctgcggtaaagctcatcagcgtggtcgtgaagcgattcacagatgtctgcctgttcatccgcgtccagctcgttgagtttctccagaagcgttaatgtctggcttctgataaagcgggccatgttaagggcggttttttcctgtttggtcactgatgcctccgtgtaagggggatttctgttcatgggggtaatgataccgatgaaacgagagaggatgctcacgatacgggttactgatgatgaacatgcccggttactggaacgttgtgagggtaaacaactggcggtatggatgcggcgggaccagagaaaaatcactcagggtcaatgccagcgcttcgttaatacagatgtaggtgttccacagggtagccagcagcatcctgcgatgcagatccggaacataatggtgcagggcgctgacttccgcgtttccagactttacgaaacacggaaaccgaagaccattcatgttgttgctcaggtcgcagacgttttgcagcagcagtcgcttcacgttcgctcgcgtatcggtgattcattctgctaaccagtaaggcaaccccgccagcctagccgggtcctcaacgacaggagcacgatcatgcgcacccgtggggccgccatgccggcgataatggcctgcttctcgccgaaacgtttggtggcgggaccagtgacgaaggcttgagcgagggcgtgcaagattccgaataccgcaagcgacaggccgatcatcgtcgcgctccagcgaaagcggtcctcgccgaaaatgacccagagcgctgccggcacctgtcctacgagttgcatgataaagaagacagtcataagtgcggcgacgatagtcatgccccgcgcccaccggaaggagctgactgggttgaaggctctcaagggcatcggtcgagatcccggtgcctaatgagtgagctaacttacattaattgcgttgcgctcactgcccgctttccagtcgggaaacctgtcgtgccagctgcattaatgaatcggccaacgcgcggggagaggcggtttgcgtattgggcgccagggtggtttttcttttcaccagtgagacgggcaacagctgattgcccttcaccgcctggccctgagagagttgcagcaagcggtccacgctggtttgccccagcaggcgaaaatcctgtttgatggtggttaacggcgggatataacatgagctgtcttcggtatcgtcgtatcccactaccgagatatccgcaccaacgcgcagcccggactcggtaatggcgcgcattgcgcccagcgccatctgatcgttggcaaccagcatcgcagtgggaacgatgccctcattcagcatttgcatggtttgttgaaaaccggacatggcactccagtcgccttcccgttccgctatcggctgaatttgattgcgagtgagatatttatgccagccagccagacgcagacgcgccgagacagaacttaatgggcccgctaacagcgcgatttgctggtgacccaatgcgaccagatgctccacgcccagtcgcgtaccgtcttcatgggagaaaataatactgttgatgggtgtctggtcagagacatcaagaaataacgccggaacattagtgcaggcagcttccacagcaatggcatcctggtcatccagcggatagttaatgatcagcccactgacgcgttgcgcgagaagattgtgcaccgccgctttacaggcttcgacgccgcttcgttctaccatcgacaccaccacgctggcacccagttgatcggcgcgagatttaatcgccgcgacaatttgcgacggcgcgtgcagggccagactggaggtggcaacgccaatcagcaacgactgtttgcccgccagttgttgtgccacgcggttgggaatgtaattcagctccgccatcgccgcttccactttttcccgcgttttcgcagaaacgtggctggcctggttcaccacgcgggaaacggtctgataagagacaccggcatactctgcgacatcgtataacgttactggtttcacattcaccaccctgaattgactctcttccgggcgctatcatgccataccgcgaaaggttttgcgccattcgatggtgtccgggatctcgacgctctcccttatgcgactcctgcattaggaagcagcccagtagtaggttgaggccgttgagcaccgccgccgcaaggaatggtgcatgcaaggagatggcgcccaacagtcccccggccacggggcctgccaccatacccacgccgaaacaagcgctcatgagcccgaagtggcgagcccgatcttccccatcggtgatgtcggcgatataggcgccagcaaccgcacctgtggcgccggtgatgccggccacgatgcgtccggcgtagaggatcgagatctcgatcccgcgaaattaatacgactcactata

SEQ ID NO: 17 - protein, 163 aa, synthetic construct
  SITE 3: note = X can be a hydrophobic amino acid including glycine, alanine and methionine
  SITE 4: note = X can be any naturally occurring amino acid
  SITE 5: note = X can be a polar and/or charged amino acid
  SITE 6: note = X can be a hydrophobic amino acid including glycine, alanine and methionine
  REGION 7..8: note = X can be any naturally occurring amino acid
  SITE 9: note = X can be a polar and/or charged amino acid
  REGION 10..11: note = X can be any naturally occurring amino acid
  SITE 12: note = X can be a polar and/or charged amino acid
  SITE 13: note = X can be any naturally occurring amino acid
  SITE 14: note = X can be a hydrophobic amino acid including glycine, alanine and methionine
  SITE 15: note = X can be any naturally occurring amino acid
  SITE 16: note = X can be a hydrophobic amino acid including glycine, alanine and methionine
  SITE 17: note = X can be any naturally occurring amino acid
  SITE 18: note = X can be a polar and/or charged amino acid
  SITE 19: note = X can be a hydrophobic amino acid including glycine, alanine and methionine
  SITE 21: note = X can be a polar and/or charged amino acid
  REGION 22..23: note = X can be any naturally occurring amino acid
  SITE 24: note = X can be a hydrophobic amino acid including glycine, alanine and methionine
  SITE 25: note = X can be any naturally occurring amino acid
  SITE 27: note = X can be any naturally occurring amino acid
  REGION 28..29: note = X can be a polar and/or charged amino acid
  SITE 30: note = X can be a hydrophobic amino acid including glycine, alanine and methionine
  SITE 31: note = X can be any naturally occurring amino acid
  SITE 33: note = X can be a polar and/or charged amino acid
  REGION 34..35: note = X can be any naturally occurring amino acid
  SITE 36: note = X can be any naturally occurring amino acid or no amino acid
  SITE 37: note = X can be a polar and/or charged amino acid
  SITE 38: note = X can be any naturally occurring amino acid
  SITE 39: note = X can be a hydrophobic amino acid including glycine, alanine and methionine
  SITE 41: note = X can be a polar and/or charged amino acid
  SITE 42: note = X can be a hydrophobic amino acid including glycine, alanine and methionine
  SITE 43: note = X can be a polar and/or charged amino acid
  SITE 44: note = X can be any naturally occurring amino acid
  SITE 45: note = X can be a hydrophobic amino acid including glycine, alanine and methionine
  SITE 46: note = X can be a polar and/or charged amino acid
  SITE 48: note = X can be a polar and/or charged amino acid
  SITE 50: note = X can be any naturally occurring amino acid or no amino acid
  SITE 51: note = X can be any naturally occurring amino acid
  SITE 52: note = X can be a hydrophobic amino acid including glycine, alanine and methionine
  SITE 54: note = X can be a polar and/or charged amino acid
  SITE 55: note = X can be a hydrophobic amino acid including glycine, alanine and methionine
  REGION 56..58: note = X can be any naturally occurring amino acid
  SITE 59: note = X can be a polar and/or charged amino acid
  SITE 61: note = X can be any naturally occurring amino acid
  SITE 62: note = X can be a polar and/or charged amino acid
  SITE 63: note = X can be any naturally occurring amino acid
  SITE 65: note = X can be any naturally occurring amino acid
  SITE 66: note = X can be a hydrophobic amino acid including glycine, alanine and methionine
  SITE 67: note = X can be a polar and/or charged amino acid
  SITE 68: note = X can be any naturally occurring amino acid
  SITE 69: note = X can be a hydrophobic amino acid including glycine, alanine and methionine
  SITE 71: note = X can be any naturally occurring amino acid
  SITE 72: note = X can be a polar and/or charged amino acid
  SITE 73: note = X can be a hydrophobic amino acid including glycine, alanine and methionine
  SITE 74: note = X can be a polar and/or charged amino acid
  SITE 75: note = X can be any naturally occurring amino acid
  SITE 76: note = X can be a hydrophobic amino acid including glycine, alanine and methionine
  REGION 77..80: note = X can be a polar and/or charged amino acid
  SITE 81: note = X can be a hydrophobic amino acid including glycine, alanine and methionine
  REGION 82..83: note = X can be any naturally occurring amino acid
  SITE 84: note = X can be a polar and/or charged amino acid
  SITE 86: note = X can be a polar and/or charged amino acid
  REGION 87..88: note = X can be a hydrophobic amino acid including glycine, alanine and methionine
  SITE 89: note = X can be any naturally occurring amino acid
  SITE 91: note = X can be a polar and/or charged amino acid
  SITE 92: note = X can be a hydrophobic amino acid including glycine, alanine and methionine
  REGION 94..96: note = X can be any naturally occurring amino acid
  SITE 97: note = X can be a hydrophobic amino acid including glycine, alanine and methionine
  REGION 98..99: note = X can be a polar and/or charged amino acid
  SITE 100: note = X can be a hydrophobic amino acid including glycine, alanine and methionine
  REGION 101..103: note = X can be any naturally occurring amino acid
  SITE 104: note = X can be a hydrophobic amino acid including glycine, alanine and methionine
  SITE 106: note = X can be a hydrophobic amino acid including glycine, alanine and methionine
  REGION 107..109: note = X can be any naturally occurring amino acid
  REGION 110..113: note = X can be any naturally occurring amino acid or no amino acid
  SITE 114: note = X can be a hydrophobic amino acid including glycine, alanine and methionine
  SITE 116: note = X can be a polar and/or charged amino acid
  SITE 117: note = X can be a hydrophobic amino acid including glycine, alanine and methionine
  SITE 118: note = X can be any naturally occurring amino acid
  SITE 119: note = X can be a polar and/or charged amino acid
  SITE 120: note = X can be any naturally occurring amino acid
  SITE 121: note = X can be a polar and/or charged amino acid
  SITE 123: note = X can be any naturally occurring amino acid
  SITE 124: note = X can be a hydrophobic amino acid including glycine, alanine and methionine
  SITE 125: note = X can be any naturally occurring amino acid
  REGION 127..131: note = X can be any naturally occurring amino acid
  SITE 132: note = X can be a hydrophobic amino acid including glycine, alanine and methionine
  SITE 133: note = X can be any naturally occurring amino acid
  SITE 134: note = X can be a polar and/or charged amino acid
  SITE 136: note = X can be a polar and/or charged amino acid
  SITE 137: note = X can be a hydrophobic amino acid including glycine, alanine and methionine
  SITE 138: note = X can be a polar and/or charged amino acid
  SITE 139: note = X can be any naturally occurring amino acid
  REGION 142..143: note = X can be a polar and/or charged amino acid
  SITE 144: note = X can be a hydrophobic amino acid including glycine, alanine and methionine
  REGION 145..146: note = X can be any naturally occurring amino acid
  REGION 147..148: note = X can be a hydrophobic amino acid including glycine, alanine and methionine
  SITE 149: note = X can be a polar and/or charged amino acid
  REGION 150..151: note = X can be a hydrophobic amino acid including glycine, alanine and methionine
  REGION 153..154: note = X can be any naturally occurring amino acid
  REGION 156..157: note = X can be any naturally occurring amino acid
  SITE 158: note = X can be a polar and/or charged amino acid
  SITE 159: note = X can be a hydrophobic amino acid including glycine, alanine and methionine
  REGION 160..163: note = X can be any naturally occurring amino acid or no amino acid
  source 1..163: note = more specific Ses iPR10 antigenic consensus sequence
MGXXXXXXXXXXXXXXXXXFXXXXXDXXXXXPXXXXXXXKXXXXXXGXGXXXGXXXXXXFXXXSXXXXXKXXXXXXXXXXXXXXYXXXXGXXLXXXXXXXXXXXKXXXXXXXXXGXXXXXXSXXXTXXXXXXXXEXXXXGKXXXXXXXXXXEXXLXXXXXXXX

SEQ ID NO: 18 - protein, 162 aa, synthetic construct
  SITE 3: note = X can be a hydrophobic amino acid including glycine, alanine and methionine
  SITE 4: note = X can be any naturally occurring amino acid
  SITE 5: note = X can be a polar and/or charged amino acid
  SITE 6: note = X can be a hydrophobic amino acid including glycine, alanine and methionine
  SITE 7: note = X can be a polar and/or charged amino acid
  SITE 8: note = X can be any naturally occurring amino acid
  SITE 9: note = X can be a polar and/or charged amino acid
  REGION 10..11: note = X can be any naturally occurring amino acid
  SITE 12: note = X can be a polar and/or charged amino acid
  SITE 13: note = X can be any naturally occurring amino acid
  SITE 14: note = X can be a hydrophobic amino acid including glycine, alanine and methionine
  SITE 15: note = X can be any naturally occurring amino acid
  SITE 16: note = X can be a hydrophobic amino acid including glycine, alanine and methionine
  SITE 17: note = X can be any naturally occurring amino acid
  SITE 18: note = X can be a polar and/or charged amino acid
  SITE 19: note = X can be a hydrophobic amino acid including glycine, alanine and methionine
  REGION 22..23: note = X can be any naturally occurring amino acid
  SITE 24: note = X can be a hydrophobic amino acid including glycine, alanine and methionine
  SITE 27: note = X can be any naturally occurring amino acid
  REGION 28..29: note = X can be a polar and/or charged amino acid
  SITE 31: note = X can be any naturally occurring amino acid
  SITE 33: note = X can be a polar and/or charged amino acid
  REGION 34..36: note = X can be a hydrophobic amino acid including glycine, alanine and methionine
  SITE 37: note = X can be a polar and/or charged amino acid
  SITE 38: note = X can be any naturally occurring amino acid
  SITE 39: note = X can be a hydrophobic amino acid including glycine, alanine and methionine
  SITE 41: note = X can be a polar and/or charged amino acid
  SITE 42: note = X can be a hydrophobic amino acid including glycine, alanine and methionine
  SITE 43: note = X can be a polar and/or charged amino acid
  REGION 44..45: note = X can be a hydrophobic amino acid including glycine, alanine and methionine
  SITE 46: note = X can be a polar and/or charged amino acid
  SITE 48: note = X can be a polar and/or charged amino acid
  SITE 50: note = X can be any naturally occurring amino acid
  SITE 51: note = X can be a hydrophobic amino acid including glycine, alanine and methionin
  SITE 53: note = X can be a polar and/or charged amino acid
  SITE 54: note = X can be a hydrophobic amino acid including glycine, alanine and methionin
  SITE 55: note = X can be a polar and/or charged amino acid
  SITE 56: note = X can be any naturally occurring amino acid
  SITE 57: note = X can be a hydrophobic amino acid including glycine, alanine and methionin
  SITE 58: note = X can be a polar and/or charged amino acid
  SITE 60: note = X can be any naturally occurring amino acid
  SITE 61: note = X can be a polar and/or charged amino acid
  SITE 62: note = X can be any naturally occurring amino acid
  SITE 64: note = X can be any naturally occurring amino acid
  SITE 65: note = X can be a hydrophobic amino acid including glycine, alanine and methionin
  SITE 66: note = X can be a polar and/or charged amino acid
  SITE 67: note = X can be any naturally occurring amino acid
  SITE 68: note = X can be a hydrophobic amino acid including glycine, alanine and methionin
  SITE 70: note = X can be any naturally occurring amino acid
  SITE 71: note = X can be a polar and/or charged amino acid
  SITE 72: note = X can be a hydrophobic amino acid including glycine, alanine and methionin
  SITE 73: note = X can be a polar and/or charged amino acid
  SITE 74: note = X can be any naturally occurring amino acid
  SITE 75: note = X can be a hydrophobic amino acid including glycine, alanine and methionin
  REGION 76..79: note = X can be a polar and/or charged amino acid
  SITE 80: note = X can be a hydrophobic amino acid including glycine, alanine and methionin
  REGION 81..82: note = X can be any naturally occurring amino acid
  SITE 83: note = X can be a polar and/or charged amino acid
  SITE 85: note = X can be a polar and/or charged amino acid
  REGION 86..87: note = X can be a hydrophobic amino acid including glycine, alanine and methionin
  SITE 88: note = X can be any naturally occurring amino acid
  REGION 93..95: note = X can be any naturally occurring amino acid
  SITE 96: note = X can be a hydrophobic amino acid including glycine, alanine and methionin
  REGION 97..98: note = X can be a polar and/or charged amino acid
  SITE 99: note = X can be a hydrophobic amino acid including glycine, alanine and methionin
  REGION 100..102: note = X can be any naturally occurring amino acid
  SITE 103: note = X can be a hydrophobic amino acid including glycine, alanine and methionin
  SITE 105: note = X can be a hydrophobic amino acid including glycine, alanine and methionin
  SITE 106: note = X can be any naturally occurring amino acid
  SITE 107: note = X can be a hydrophobic amino acid including glycine, alanine and methionin
  SITE 108: note = X can be any naturally occurring amino acid
  REGION 109..112: note = X can be any naturally occurring amino acid or no amino acid
  SITE 113: note = X can be a hydrophobic amino acid including glycine, alanine and methionin
  SITE 115: note = X can be a polar and/or charged amino acid
  SITE 116: note = X can be a hydrophobic amino acid including glycine, alanine and methionin
  REGION 117..118: note = X can be a polar and/or charged amino acid
  SITE 119: note = X can be any naturally occurring amino acid
  SITE 120: note = X can be a polar and/or charged amino acid
  SITE 122: note = X can be any naturally occurring amino acid
  SITE 123: note = X can be a hydrophobic amino acid including glycine, alanine and methionin
  SITE 124: note = X can be any naturally occurring amino acid
  REGION 126..130: note = X can be any naturally occurring amino acid
  SITE 131: note = X can be a hydrophobic amino acid including glycine, alanine and methionine
  SITE 132: note = X can be any naturally occurring amino acid
  SITE 133: note = X can be a polar and/or charged amino acid
  SITE 135: note = X can be a polar and/or charged amino acid
  SITE 136: note = X can be a hydrophobic amino acid including glycine, alanine and methionine
  SITE 137: note = X can be a polar and/or charged amino acid
  SITE 138: note = X can be any naturally occurring amino acid
  REGION 141..142: note = X can be a polar and/or charged amino acid
  SITE 143: note = X can be a hydrophobic amino acid including glycine, alanine and methionine
  REGION 144..145: note = X can be any naturally occurring amino acid
  REGION 146..147: note = X can be a hydrophobic amino acid including glycine, alanine and methionine
  SITE 148: note = X can be a polar and/or charged amino acid
  REGION 149..150: note = X can be a hydrophobic amino acid including glycine, alanine and methionine
  REGION 152..153: note = X can be any naturally occurring amino acid
  REGION 155..156: note = X can be any naturally occurring amino acid
  SITE 157: note = X can be a polar and/or charged amino acid
  SITE 158: note = X can be a hydrophobic amino acid including glycine, alanine and methionine
  REGION 159..162: note = X can be any naturally occurring amino acid or no amino acid
  source 1..162: note = even more specific iPR10 antigenic consensus sequence
MGXXXXXXXXXXXXXXXXXFKXXXLDXXXLXPXXXXXXXKXXXXXXGXGXXGXXXXXXFXXXSXXXXXKXXXXXXXXXXXXXXYXXXXGDALXXXXXXXXXXXKXXXXXXXXXGXXXXXXSXXXTXXXXXXXXEXXXXGKXXXXXXXXXXEXXLXXXXXXXX

SEQ ID NO: 19 - protein, 179 aa, synthetic construct
  source 1..179: note = sequence of variant of Ses iPR10-2, His tagged
MSHHHHHHHHLEVLFQGPSMGVLTYTEEHTSAVPPARIFKASVLDADNLIPKLLPQAIKSMEILEGTGGPGTIKQICFAEGSTYKSAKHRIDEIDEENYTYNYTVIEGDALTDKLESITHEVKIEAAPDGGTICKVTSTYHTKGDFALKEEKIKAGKERALGVYKAVEAYLLANPDAYA

SEQ ID NO: 20 - protein, 175 aa, synthetic construct
  source 1..175: note = sequence of variant of Ses iPR10-5, His tagged
MSHHHHHHHHLEVLFQGPSMGVLTYDIEIPSSVPPARMFKAVVLDADNLIPKLLPQAIKSVEILEGDGGPGTIKIIHFAEGSQYKSAKHRIDEIDEENYTYSYTVIEGDALAGVLESITHHVKIEPTEDGGCICKNTSTYHTKGDVEITEEKIKAGKERAMQMLKAVEAYLQANP

SEQ ID NO: 21 - protein, 179 aa, synthetic construct
  source 1..179: note = sequence of variant of Ses iPR10-6, His tagged
MSHHHHHHHHLEVLFQGPSMGVLTYEDELISPVPPARLFKALVLDADNLIPKLLPQAIKSFEILEGHGGPGTIKLITFAEGSPYKSAKHRIDEIDEENYTYKYTVIEGDALGEDLESITHGVKIEVGADGGSICKTTSTYHTKGDDHVIEEKIKAGKERAKAIFKAVEAYLHANPHEYN

SEQ ID NO: 22 - DNA, 5784 bp, synthetic construct
  source 1..5784: mol_type = other DNA; note = vector sequence, used to express sequence of variant of Ses iPR10-2
ggggaattgtgagcggataacaattcccctctagaaataattttgtttaactttaagaaggagatataccatgagccatcatcatcatcatcatcatcatttggaagtgctgtttcagggtccatccatgggtgtactcacttacactgaggagcacacatctgcagttccgccagcaagaatcttcaaagcttcagtcctggacgccgacaacttgatcccaaagcttcttccacaggccatcaagagcatggaaattctggaaggcactggcggtcctgggaccatcaaacagatctgttttgctgaaggtagcacttataaaagtgcgaagcatcggattgatgagattgatgaagagaactatacgtataattacacagtaattgaaggcgatgcgttgacagacaaacttgagagcatcactcatgaggtgaagatagaggcagcgcccgatggtggcacaatctgtaaggtgacgagcacgtatcacacgaaaggcgattttgctctgaaagaggaaaagattaaagcagggaaggagagggcgcttggggtatacaaggcagttgaggcttacctcctcgccaaccccgatgcctatgcttaatgatcgagtaagtcgagcaccaccaccaccaccactgagatccggctgctaacaaagcccgaaaggaagctgagttggctgctgccaccgctgagcaataactagcataaccccttggggcctctaaacgggtcttgaggggttttttgctgaaaggaggaactatatccggattggcgaatgggacgcgccctgtagcggcgcattaagcgcggcgggtgtggtggttacgcgcagcgtgaccgctacacttgccagcgccctagcgcccgctcctttcgctttcttcccttcctttctcgccacgttcgccggctttccccgtcaagctctaaatcgggggctccctttagggttccgatttagtgctttacggcacctcgaccccaaaaaacttgattagggtgatggttcacgtagtgggccatcgccctgatagacggtttttcgccctttgacgttggagtccacgttctttaatagtggactcttgttccaaactggaacaacactcaaccctatctcggtctattcttttgatttataagggattttgccgatttcggcctattggttaaaaaatgagctgatttaacaaaaatttaacgcgaattttaacaaaatattaacgtttacaatttcaggtggcacttttcggggaaatgtgcgcggaacccctatttgtttatttttctaaatacattcaaatatgtatccgctcatgaattaattcttagaaaaactcatcgagcatcaaatgaaactgcaatttattcatatcaggattatcaataccatatttttgaaaaagccgtttctgtaatgaaggagaaaactcaccgaggcagttccataggatggcaagatcctggtatcggtctgcgattccgactcgtccaacatcaatacaacctattaatttcccctcgtcaaaaataaggttatcaagtgagaaatcaccatgagtgacgactgaatccggtgagaatggcaaaagtttatgcatttctttccagacttgttcaacaggccagccattacgctcgtcatcaaaatcactcgcatcaaccaaaccgttattcattcgtgattgcgcctgagcgagacgaaatacgcgatcgctgttaaaaggacaattacaaacaggaatcgaatgcaaccggcgcaggaacactgccagcgcatcaacaatattttcacctgaatcaggatattcttctaatacctggaatgctgttttcccggggatcgcagtggtgagtaaccatgcatcatcaggagtacggataaaatgcttgatggtcggaagaggcataaattccgtcagccagtttagtctgaccatctcatctgtaacatcattggcaacgctacctttgccatgtttcagaaacaactctggcgcatcgggcttcccatacaatcgatagattgtcgcacctgattgcccgacattatcgcgagcccatttatacccatataaatcagcatccatgttggaatttaatcgcggcctagagcaagacgtttcccgttgaatatggctcataacaccccttgtattactgtttatgtaagcagacagttttattgttcatgaccaaaatcccttaacgtgagttttcgttccactgagcgtcagaccccgtagaaaagatcaaaggatcttcttgagatcctttttttctgcgcgtaatctgctgcttgcaaacaaaaaaaccaccgctaccagcggtggtttgtttgccggatcaagagctaccaactctttttccgaaggtaactggcttcagcagagcgcagataccaaatactgtccttctagtgtagccgtagttaggccaccacttcaagaactctgtagcaccgcctacatacctcgctctgctaatcctgttaccagtggctgctgccagtggcgataagtcgtgtcttaccgggttggactcaagacgatagttaccggataaggcgcagcggtcgggctgaacggggggttcgtgcacacagcccagcttggagcgaacgacctacaccgaactgagatacctacagcgtgagctatgagaaagcgccacgcttcccgaagggagaaaggcggacaggtatccggtaagcggcagggtcggaacaggagagcgcacgagggagcttccagggggaaacgcctggtatctttatagtcctgtcgggtttcgccacctctgacttgagcgtcgatttttgtgatgctcgtcaggggggcggagcctatggaaaaacgccagcaacgcggcctttttacggttcctggccttttgctggccttttgctcacatgttctttcctgcgttatcccctgattctgtggataaccgtattaccgcctttgagtgagctgataccgctcgccgcagccgaacgaccgagcgcagcgagtcagtgagcgaggaagcggaagagcgcctgatgcggtattttctccttacgcatctgtgcggtatttcacaccgcatatatggtgcactctcagtacaatctgctctgatgccgcatagttaagccagtatacactccgctatcgctacgtgactgggtcatggctgcgccccgacacccgccaacacccgctgacgcgccctgacgggcttgtctgctcccggcatccgcttacagacaagctgtgaccgtctccgggagctgcatgtgtcagaggttttcaccgtcatcaccgaaacgcgcgaggcagctgcggtaaagctcatcagcgtggtcgtgaagcgattcacagatgtctgcctgttcatccgcgtccagctcgttgagtttctccagaagcgttaatgtctggcttctgataaagcgggccatgttaagggcggttttttcctgtttggtcactgatgcctccgtgtaagggggatttctgttcatgggggtaatgataccgatgaaacgagagaggatgctcacgatacgggttactgatgatgaacatgcccggttactggaacgttgtgagggtaaacaactggcggtatggatgcggcgggaccagagaaaaatcactcagggtcaatgccagcgcttcgttaatacagatgtaggtgttccacagggtagccagcagcatcctgcgatgcagatccggaacataatggtgcagggcgctgacttccgcgtttccagactttacgaaacacggaaaccgaagaccattcatgttgttgctcaggtcgcagacgttttgcagcagcagtcgcttcacgttcgctcgcgtatcggtgattcattctgctaaccagtaaggcaaccccgccagcctagccgggtcctcaacgacaggagcacgatcatgcgcacccgtggggccgccatgccggcgataatggcctgcttctcgccgaaacgtttggtggcgggaccagtgacgaaggcttgagcgagggcgtgcaagattccgaataccgcaagcgacaggccgatcatcgtcgcgctccagcgaaagcggtcctcgccgaaaatgacccagagcgctgccggcacctgtcctacgagttgcatgataaagaagacagtcataagtgcggcgacgatagtcatgccccgcgcccaccggaaggagctgactgggttgaaggctctcaagggcatcggtcgagatcccggtgcctaatgagtgagctaacttacattaattgcgttgcgctcactgcccgctttccagtcgggaaacctgtcgtgccagctgcattaatgaatcggccaacgcgcggggagaggcggtttgcgtattgggcgccagggtggtttttcttttcaccagtgagacgggcaacagctgattgcccttcaccgcctggccctgagagagttgcagcaagcggtccacgctggtttgccccagcaggcgaaaatcctgtttgatggtggttaacggcgggatataacatgagctgtcttcggtatcgtcgtatcccactaccgagatatccgcaccaacgcgcagcccggactcggtaatggcgcgcattgcgcccagcgccatctgatcgttggcaaccagcatcgcagtgggaacgatgccctcattcagcatttgcatggtttgttgaaaaccggacatggcactccagtcgccttcccgttccgctatcggctgaatttgattgcgagtgagatatttatgccagccagccagacgcagacgcgccgagacagaacttaatgggcccgctaacagcgcgatttgctggtgacccaatgcgaccagatgctccacgcccagtcgcgtaccgtcttcatgggagaaaataatactgttgatgggtgtctggtcagagacatcaagaaataacgccggaacattagtgcaggcagcttccacagcaatggcatcctggtcatccagcggatagttaatgatcagcccactgacgcgttgcgcgagaagattgtgcaccgccgctttacaggcttcgacgccgcttcgttctaccatcgacaccaccacgctggcacccagttgatcggcgcgagatttaatcgccgcgacaatttgcgacggcgcgtgcagggccagactggaggtggcaacgccaatcagcaacgactgtttgcccgccagttgttgtgccacgcggttgggaatgtaattcagctccgccatcgccgcttccactttttcccgcgttttcgcagaaacgtggctggcctggttcaccacgcgggaaacggtctgataagagacaccggcatactctgcgacatcgtataacgttactggtttcacattcaccaccctgaattgactctcttccgggcgctatcatgccataccgcgaaaggttttgcgccattcgatggtgtccgggatctcgacgctctcccttatgcgactcctgcattaggaagcagcccagtagtaggttgaggccgttgagcaccgccgccgcaaggaatggtgcatgcaaggagatggcgcccaacagtcccccggccacggggcctgccaccatacccacgccgaaacaagcgctcatgagcccgaagtggcgagcccgatcttccccatcggtgatgtcggcgatataggcgccagcaaccgcacctgtggcgccggtgatgccggccacgatgcgtccggcgtagaggatcgagatctcgatcccgcgaaattaatacgactcactata

SEQ ID NO: 23 - DNA, 5772 bp, synthetic construct
  source 1..5772: mol_type = other DNA; note = vector sequence, used to express sequence of variant of Ses iPR10-5
ggggaattgtgagcggataacaattcccctctagaaataattttgtttaactttaagaaggagatataccatgagccatcatcatcatcatcatcatcatttggaagtgctgtttcagggtccatccatgggtgtactcacttacgatattgagattccttcctcagttccgccagcaagaatgtttaaggccgttgtcctcgatgcggataaccttattcctaaacttcttccacaggccatcaagagcgttgaaatcttggaaggagatggtggtcctgggaccatcaaaatcatccattttgctgagggcagccagtataagagcgcaaagcaccgtattgatgagattgatgaagagaactatacgtatagctacaccgttattgagggtgacgcactggccggagttcttgaatccatcactcatcatgtcaagattgagccgactgaagatggaggatgcatatgcaagaacaccagcacgtaccacaccaagggcgacgttgagatcaccgaagagaagatcaaggcagggaaggagagggcgatgcagatgctcaaggccgttgaagcttacctccaagctaatccataatgatcgagtaagtcgagcaccaccaccaccaccactgagatccggctgctaacaaagcccgaaaggaagctgagttggctgctgccaccgctgagcaataactagcataaccccttggggcctctaaacgggtcttgaggggttttttgctgaaaggaggaactatatccggattggcgaatgggacgcgccctgtagcggcgcattaagcgcggcgggtgtggtggttacgcgcagcgtgaccgctacacttgccagcgccctagcgcccgctcctttcgctttcttcccttcctttctcgccacgttcgccggctttccccgtcaagctctaaatcgggggctccctttagggttccgatttagtgctttacggcacctcgaccccaaaaaacttgattagggtgatggttcacgtagtgggccatcgccctgatagacggtttttcgccctttgacgttggagtccacgttctttaatagtggactcttgttccaaactggaacaacactcaaccctatctcggtctattcttttgatttataagggattttgccgatttcggcctattggttaaaaaatgagctgatttaacaaaaatttaacgcgaattttaacaaaatattaacgtttacaatttcaggtggcacttttcggggaaatgtgcgcggaacccctatttgtttatttttctaaatacattcaaatatgtatccgctcatgaattaattcttagaaaaactcatcgagcatcaaatgaaactgcaatttattcatatcaggattatcaataccatatttttgaaaaagccgtttctgtaatgaaggagaaaactcaccgaggcagttccataggatggcaagatcctggtatcggtctgcgattccgactcgtccaacatcaatacaacctattaatttcccctcgtcaaaaataaggttatcaagtgagaaatcaccatgagtgacgactgaatccggtgagaatggcaaaagtttatgcatttctttccagacttgttcaacaggccagccattacgctcgtcatcaaaatcactcgcatcaaccaaaccgttattcattcgtgattgcgcctgagcgagacgaaatacgcgatcgctgttaaaaggacaattacaaacaggaatcgaatgcaaccggcgcaggaacactgccagcgcatcaacaatattttcacctgaatcaggatattcttctaatacctggaatgctgttttcccggggatcgcagtggtgagtaaccatgcatcatcaggagtacggataaaatgcttgatggtcggaagaggcataaattccgtcagccagtttagtctgaccatctcatctgtaacatcattggcaacgctacctttgccatgtttcagaaacaactctggcgcatcgggcttcccatacaatcgatagattgtcgcacctgattgcccgacattatcgcgagcccatttatacccatataaatcagcatccatgttggaatttaatcgcggcctagagcaagacgtttcccgttgaatatggctcataacaccccttgtattactgtttatgtaagcagacagttttattgttcatgaccaaaatcccttaacgtgagttttcgttccactgagcgtcagaccccgtagaaaagatcaaaggatcttcttgagatcctttttttctgcgcgtaatctgctgcttgcaaacaaaaaaaccaccgctaccagcggtggtttgtttgccggatcaagagctaccaactctttttccgaaggtaactggcttcagcagagcgcagataccaaatactgtccttctagtgtagccgtagttaggccaccacttcaagaactctgtagcaccgcctacatacctcgctctgctaatcctgttaccagtggctgctgccagtggcgataagtcgtgtcttaccgggttggactcaagacgatagttaccggataaggcgcagcggtcgggctgaacggggggttcgtgcacacagcccagcttggagcgaacgacctacaccgaactgagatacctacagcgtgagctatgagaaagcgccacgcttcccgaagggagaaaggcggacaggtatccggtaagcggcagggtcggaacaggagagcgcacgagggagcttccagggggaaacgcctggtatctttatagtcctgtcgggtttcgccacctctgacttgagcgtcgatttttgtgatgctcgtcaggggggcggagcctatggaaaaacgccagcaacgcggcctttttacggttcctggccttttgctggccttttgctcacatgttctttcctgcgttatcccctgattctgtggataaccgtattaccgcctttgagtgagctgataccgctcgccgcagccgaacgaccgagcgcagcgagtcagtgagcgaggaagcggaagagcgcctgatgcggtattttctccttacgcatctgtgcggtatttcacaccgcatatatggtgcactctcagtacaatctgctctgatgccgcatagttaagccagtatacactccgctatcgctacgtgactgggtcatggctgcgccccgacacccgccaacacccgctgacgcgccctgacgggcttgtctgctcccggcatccgcttacagacaagctgtgaccgtctccgggagctgcatgtgtcagaggttttcaccgtcatcaccgaaacgcgcgaggcagctgcggtaaagctcatcagcgtggtcgtgaagcgattcacagatgtctgcctgttcatccgcgtccagctcgttgagtttctccagaagcgttaatgtctggcttctgataaagcgggccatgttaagggcggttttttcctgtttggtcactgatgcctccgtgtaagggggatttctgttcatgggggtaatgataccgatgaaacgagagaggatgctcacgatacgggttactgatgatgaacatgcccggttactggaacgttgtgagggtaaacaactggcggtatggatgcggcgggaccagagaaaaatcactcagggtcaatgccagcgcttcgttaatacagatgtaggtgttccacagggtagccagcagcatcctgcgatgcagatccggaacataatggtgcagggcgctgacttccgcgtttccagactttacgaaacacggaaaccgaagaccattcatgttgttgctcaggtcgcagacgttttgcagcagcagtcgcttcacgttcgctcgcgtatcggtgattcattctgctaaccagtaaggcaaccccgccagcctagccgggtcctcaacgacaggagcacgatcatgcgcacccgtggggccgccatgccggcgataatggcctgcttctcgccgaaacgtttggtggcgggaccagtgacgaaggcttgagcgagggcgtgcaagattccgaataccgcaagcgacaggccgatcatcgtcgcgctccagcgaaagcggtcctcgccgaaaatgacccagagcgctgccggcacctgtcctacgagttgcatgataaagaagacagtcataagtgcggcgacgatagtcatgccccgcgcccaccggaaggagctgactgggttgaaggctctcaagggcatcggtcgagatcccggtgcctaatgagtgagctaacttacattaattgcgttgcgctcactgcccgctttccagtcgggaaacctgtcgtgccagctgcattaatgaatcggccaacgcgcggggagaggcggtttgcgtattgggcgccagggtggtttttcttttcaccagtgagacgggcaacagctgattgcccttcaccgcctggccctgagagagttgcagcaagcggtccacgctggtttgccccagcaggcgaaaatcctgtttgatggtggttaacggcgggatataacatgagctgtcttcggtatcgtcgtatcccactaccgagatatccgcaccaacgcgcagcccggactcggtaatggcgcgcattgcgcccagcgccatctgatcgttggcaaccagcatcgcagtgggaacgatgccctcattcagcatttgcatggtttgttgaaaaccggacatggcactccagtcgccttcccgttccgctatcggctgaatttgattgcgagtgagatatttatgccagccagccagacgcagacgcgccgagacagaacttaatgggcccgctaacagcgcgatttgctggtgacccaatgcgaccagatgctccacgcccagtcgcgtaccgtcttcatgggagaaaataatactgttgatgggtgtctggtcagagacatcaagaaataacgccggaacattagtgcaggcagcttccacagcaatggcatcctggtcatccagcggatagttaatgatcagcccactgacgcgttgcgcgagaagattgtgcaccgccgctttacaggcttcgacgccgcttcgttctaccatcgacaccaccacgctggcacccagttgatcggcgcgagatttaatcgccgcgacaatttgcgacggcgcgtgcagggccagactggaggtggcaacgccaatcagcaacgactgtttgcccgccagttgttgtgccacgcggttgggaatgtaattcagctccgccatcgccgcttccactttttcccgcgttttcgcagaaacgtggctggcctggttcaccacgcgggaaacggtctgataagagacaccggcatactctgcgacatcgtataacgttactggtttcacattcaccaccctgaattgactctcttccgggcgctatcatgccataccgcgaaaggttttgcgccattcgatggtgtccgggatctcgacgctctcccttatgcgactcctgcattaggaagcagcccagtagtaggttgaggccgttgagcaccgccgccgcaaggaatggtgcatgcaaggagatggcgcccaacagtcccccggccacggggcctgccaccatacccacgccgaaacaagcgctcatgagcccgaagtggcgagcccgatcttccccatcggtgatgtcggcgatataggcgccagcaaccgcacctgtggcgccggtgatgccggccacgatgcgtccggcgtagaggatcgagatctcgatcccgcgaaattaatacgactcactata

SEQ ID NO: 24 - DNA, 5784 bp, synthetic construct
  source 1..5784: mol_type = other DNA; note = vector sequence, used to express sequence of variant of Ses iPR10-6
ggggaattgtgagcggataacaattcccctctagaaataattttgtttaactttaagaaggagatataccatgagccatcatcatcatcatcatcatcatttggaagtgctgtttcagggtccatccatgggtgtactcacttacgaggatgaactgatctccccagtcccaccagctaggttgtttaaggcactcgttctggacgcagacaacctcattcctaagcttctgccacaagccattaagagctttgaaatcctagagggccatggaggacctggaaccatcaaattgatcacttttgctgaagggagtccttacaagagcgcaaagcatcgtattgatgaaattgacgaggaaaattacacctacaagtacaccgtgatagaaggtgatgctcttggggaagatcttgaatccatcacgcacggtgtcaagatcgaagtcggggcggatggaggatctatctgcaaaaccaccagcacataccacaccaaaggggacgatcatgttatagaagaaaagatcaaggctggcaaagagagggcaaaggcaattttcaaggctgttgaggcatacctccatgcaaaccctcatgaatacaactaatgatcgagtaagtcgagcaccaccaccaccaccactgagatccggctgctaacaaagcccgaaaggaagctgagttggctgctgccaccgctgagcaataactagcataaccccttggggcctctaaacgggtcttgaggggttttttgctgaaaggaggaactatatccggattggcgaatgggacgcgccctgtagcggcgcattaagcgcggcgggtgtggtggttacgcgcagcgtgaccgctacacttgccagcgccctagcgcccgctcctttcgctttcttcccttcctttctcgccacgttcgccggctttccccgtcaagctctaaatcgggggctccctttagggttccgatttagtgctttacggcacctcgaccccaaaaaacttgattagggtgatggttcacgtagtgggccatcgccctgatagacggtttttcgccctttgacgttggagtccacgttctttaatagtggactcttgttccaaactggaacaacactcaaccctatctcggtctattcttttgatttataagggattttgccgatttcggcctattggttaaaaaatgagctgatttaacaaaaatttaacgcgaattttaacaaaatattaacgtttacaatttcaggtggcacttttcggggaaatgtgcgcggaacccctatttgtttatttttctaaatacattcaaatatgtatccgctcatgaattaattcttagaaaaactcatcgagcatcaaatgaaactgcaatttattcatatcaggattatcaataccatatttttgaaaaagccgtttctgtaatgaaggagaaaactcaccgaggcagttccataggatggcaagatcctggtatcggtctgcgattccgactcgtccaacatcaatacaacctattaatttcccctcgtcaaaaataaggttatcaagtgagaaatcaccatgagtgacgactgaatccggtgagaatggcaaaagtttatgcatttctttccagacttgttcaacaggccagccattacgctcgtcatcaaaatcactcgcatcaaccaaaccgttattcattcgtgattgcgcctgagcgagacgaaatacgcgatcgctgttaaaaggacaattacaaacaggaatcgaatgcaaccggcgcaggaacactgccagcgcatcaacaatattttcacctgaatcaggatattcttctaatacctggaatgctgttttcccggggatcgcagtggtgagtaaccatgcatcatcaggagtacggataaaatgcttgatggtcggaagaggcataaattccgtcagccagtttagtctgaccatctcatctgtaacatcattggcaacgctacctttgccatgtttcagaaacaactctggcgcatcgggcttcccatacaatcgatagattgtcgcacctgattgcccgacattatcgcgagcccatttatacccatataaatcagcatccatgttggaatttaatcgcggcctagagcaagacgtttcccgttgaatatggctcataacaccccttgtattactgtttatgtaagcagacagttttattgttcatgaccaaaatcccttaacgtgagttttcgttccactgagcgtcagaccccgtagaaaagatcaaaggatcttcttgagatcctttttttctgcgcgtaatctgctgcttgcaaacaaaaaaaccaccgctaccagcggtggtttgtttgccggatcaagagctaccaactctttttccgaaggtaactggcttcagcagagcgcagataccaaatactgtccttctagtgtagccgtagttaggccaccacttcaagaactctgtagcaccgcctacatacctcgctctgctaatcctgttaccagtggctgctgccagtggcgataagtcgtgtcttaccgggttggactcaagacgatagttaccggataaggcgcagcggtcgggctgaacggggggttcgtgcacacagcccagcttggagcgaacgacctacaccgaactgagatacctacagcgtgagctatgagaaagcgccacgcttcccgaagggagaaaggcggacaggtatccggtaagcggcagggtcggaacaggagagcgcacgagggagcttccagggggaaacgcctggtatctttatagtcctgtcgggtttcgccacctctgacttgagcgtcgatttttgtgatgctcgtcaggggggcggagcctatggaaaaacgccagcaacgcggcctttttacggttcctggccttttgctggccttttgctcacatgttctttcctgcgttatcccctgattctgtggataaccgtattaccgcctttgagtgagctgataccgctcgccgcagccgaacgaccgagcgcagcgagtcagtgagcgaggaagcggaagagcgcctgatgcggtattttctccttacgcatctgtgcggtatttcacaccgcatatatggtgcactctcagtacaatctgctctgatgccgcatagttaagccagtatacactccgctatcgctacgtgactgggtcatggctgcgccccgacacccgccaacacccgctgacgcgccctgacgggcttgtctgctcccggcatccgcttacagacaagctgtgaccgtctccgggagctgcatgtgtcagaggttttcaccgtcatcaccgaaacgcgcgaggcagctgcggtaaagctcatcagcgtggtcgtgaagcgattcacagatgtctgcctgttcatccgcgtccagctcgttgagtttctccagaagcgttaatgtctggcttctgataaagcgggccatgttaagggcggttttttcctgtttggtcactgatgcctccgtgtaagggggatttctgttcatgggggtaatgataccgatgaaacgagagaggatgctcacgatacgggttactgatgatgaacatgcccggttactggaacgttgtgagggtaaacaactggcggtatggatgcggcgggaccagagaaaaatcactcagggtcaatgccagcgcttcgttaatacagatgtaggtgttccacagggtagccagcagcatcctgcgatgcagatccggaacataatggtgcagggcgctgacttccgcgtttccagactttacgaaacacggaaaccgaagaccattcatgttgttgctcaggtcgcagacgttttgcagcagcagtcgcttcacgttcgctcgcgtatcggtgattcattctgctaaccagtaaggcaaccccgccagcctagccgggtcctcaacgacaggagcacgatcatgcgcacccgtggggccgccatgccggcgataatggcctgcttctcgccgaaacgtttggtggcgggaccagtgacgaaggcttgagcgagggcgtgcaagattccgaataccgcaagcgacaggccgatcatcgtcgcgctccagcgaaagcggtcctcgccgaaaatgacccagagcgctgccggcacctgtcctacgagttgcatgataaagaagacagtcataagtgcggcgacgatagtcatgccccgcgcccaccggaaggagctgactgggttgaaggctctcaagggcatcggtcgagatcccggtgcctaatgagtgagctaacttacattaattgcgttgcgctcactgcccgctttccagtcgggaaacctgtcgtgccagctgcattaatgaatcggccaacgcgcggggagaggcggtttgcgtattgggcgccagggtggtttttcttttcaccagtgagacgggcaacagctgattgcccttcaccgcctggccctgagagagttgcagcaagcggtccacgctggtttgccccagcaggcgaaaatcctgtttgatggtggttaacggcgggatataacatgagctgtcttcggtatcgtcgtatcccactaccgagatatccgcaccaacgcgcagcccggactcggtaatggcgcgcattgcgcccagcgccatctgatcgttggcaaccagcatcgcagtgggaacgatgccctcattcagcatttgcatggtttgttgaaaaccggacatggcactccagtcgccttcccgttccgctatcggctgaatttgattgcgagtgagatatttatgccagccagccagacgcagacgcgccgagacagaacttaatgggcccgctaacagcgcgatttgctggtgacccaatgcgaccagatgctccacgcccagtcgcgtaccgtcttcatgggagaaaataatactgttgatgggtgtctggtcagagacatcaagaaataacgccggaacattagtgcaggcagcttccacagcaatggcatcctggtcatccagcggatagttaatgatcagcccactgacgcgttgcgcgagaagattgtgcaccgccgctttacaggcttcgacgccgcttcgttctaccatcgacaccaccacgctggcacccagttgatcggcgcgagatttaatcgccgcgacaatttgcgacggcgcgtgcagggccagactggaggtggcaacgccaatcagcaacgactgtttgcccgccagttgttgtgccacgcggttgggaatgtaattcagctccgccatcgccgcttccactttttcccgcgttttcgcagaaacgtggctggcctggttcaccacgcgggaaacggtctgataagagacaccggcatactctgcgacatcgtataacgttactggtttcacattcaccaccctgaattgactctcttccgggcgctatcatgccataccgcgaaaggttttgcgccattcgatggtgtccgggatctcgacgctctcccttatgcgactcctgcattaggaagcagcccagtagtaggttgaggccgttgagcaccgccgccgcaaggaatggtgcatgcaaggagatggcgcccaacagtcccccggccacggggcctgccaccatacccacgccgaaacaagcgctcatgagcccgaagtggcgagcccgatcttccccatcggtgatgtcggcgatataggcgccagcaaccgcacctgtggcgccggtgatgccggccacgatgcgtccggcgtagaggatcgagatctcgatcccgcgaaattaatacgactcactata

SEQ ID NO: 25 - protein, 160 aa, synthetic construct
  source 1..160: note = sequence of variant of Ses iPR10-2
MGVLTYTEEHTSAVPPARIFKASVLDADNLIPKLLPQAIKSMEILEGTGGPGTIKQICFAEGSTYKSAKHRIDEIDEENYTYNYTVIEGDALTDKLESITHEVKIEAAPDGGTICKVTSTYHTKGDFALKEEKIKAGKERALGVYKAVEAYLLANPDAYA

SEQ ID NO: 26 - protein, 156 aa, synthetic construct
  source 1..156: note = sequence of variant of Ses iPR10-5
MGVLTYDIEIPSSVPPARMFKAVVLDADNLIPKLLPQAIKSVEILEGDGGPGTIKIIHFAEGSQYKSAKHRIDEIDEENYTYSYTVIEGDALAGVLESITHHVKIEPTEDGGCICKNTSTYHTKGDVEITEEKIKAGKERAMQMLKAVEAYLQANP

SEQ ID NO: 27 - protein, 160 aa, synthetic construct
  source 1..160: note = sequence of variant of Ses iPR10-6
MGVLTYEDELISPVPPARLFKALVLDADNLIPKLLPQAIKSFEILEGHGGPGTIKLITFAEGSPYKSAKHRIDEIDEENYTYKYTVIEGDALGEDLESITHGVKIEVGADGGSICKTTSTYHTKGDDHVIEEKIKAGKERAKAIFKAVEAYLHANPHEYN

SEQ ID NO: 28 - protein, 159 aa, synthetic construct
  source 1..159: note = Ses iPR10-2/5/6 consensus sequence
  REGION 2..7: note = X can be any naturally occuring amino acid
  REGION 9..10: note = X can be any naturally occuring amino acid
  REGION 12..18: note = X can be any naturally occuring amino acid
  REGION 21..23: note = X can be any naturally occuring amino acid
  REGION 26..28: note = X can be any naturally occuring amino acid
  REGION 33..34: note = X can be any naturally occuring amino acid
  REGION 36..38: note = X can be any naturally occuring amino acid
  REGION 40..45: note = X can be any naturally occuring amino acid
  REGION 49..50: note = X can be any naturally occuring amino acid
  SITE 47: note = X can be any naturally occuring amino acid
  REGION 52..53: note = X can be any naturally occuring amino acid
  REGION 59..60: note = X can be any naturally occuring amino acid
  REGION 55..57: note = X can be any naturally occuring amino acid
  REGION 63..67: note = X can be any naturally occuring amino acid
  SITE 69: note = X can be any naturally occuring amino acid
  SITE 71: note = X can be any naturally occuring amino acid
  REGION 73..76: note = X can be any naturally occuring amino acid
  REGION 78..82: note = X can be any naturally occuring amino acid
  REGION 84..87: note = X can be any naturally occuring amino acid
  REGION 92..98: note = X can be any naturally occuring amino acid
  REGION 100..102: note = X can be any naturally occuring amino acid
  REGION 104..109: note = X can be any naturally occuring amino acid
  REGION 112..114: note = X can be any naturally occuring amino acid
  REGION 116..117: note = X can be any naturally occuring amino acid
  REGION 119..121: note = X can be any naturally occuring amino acid
  REGION 125..130: note = X can be any naturally occuring amino acid
  REGION 132..133: note = X can be any naturally occuring amino acid
  REGION 139..144: note = X can be any naturally occuring amino acid
  SITE 135: note = X can be any naturally occuring amino acid
  REGION 146..147: note = X can be any naturally occuring amino acid
  REGION 149..150: note = X can be any naturally occuring amino acid
  REGION 152..159: note = X can be any naturally occuring amino acid
GXXXXXXEXXSXXXXXXXFKXXXLDXXXLIPKXXPXXXKXXXXXXGXGXXGXXKXXXFXXGSXXXXXKXRXDXXXXEXXXXXYXXXXGDALXXXXXXXTXXXKXXXXXXGGXXXKXXSXXXTKGXXXXXXEXXKXGKEXXXXXXKXXEXXLXXXXXXXX